European Patent Application EP 4 414 385 A2, published August 14, 2024. Title: POLYOMAVIRUS NEUTRALISING ANTIBODIES. Applicant: NOVARTIS AG. Application EP. The sequence listing filed with the application follows.

SEQUENCE LISTING (538 sequences)

SEQ ID NO: 1 - protein, 362 aa, Polyomavirus
MAPTKRKGECPGAAPKKPKEPVQVPKLLIKGGVEVLEVKTGVDAITEVECFLNPEMGDPDENLRGFSLKLSAENDFSSDSPERKMLPCYSTARIPLPNLNEDLTCGNLLMWEAVTVQTEVIGITSMLNLHAGSQKVHEHGGGKPIQGSNFHFFAVGGDPLEMQGVLMNYRTKYPEGTITPKNPTAQSQVMNTDHKAYLDKNNAYPVECWIPDPSRNENTRYFGTFTGGENVPPVLHVTNTATTVLLDEQGVGPLCKADSLYVSAADICGLFTNSSGTQQWRGLARYFKIRLRKRSVKNPYPISFLLSDLINRRTQRVDGQPMYGMESQVEEVRVFDGTERLPGDPDMIRYIDKQGQLQTKML

SEQ ID NO: 2 - protein, 362 aa, Polyomavirus
MAPTKRKGECPGAAPKKPKEPVQVPKLLIKGGVEVLEVKTGVDAITEVECFLNPEMGDPDDNLRGYSLKLTAENAFDSDSPDKKMLPCYSTARIPLPNLNEDLTCGNLLMWEAVTVKTEVIGITSMLNLHAGSQKVHENGGGKPVQGSNFHFFAVGGDPLEMQGVLMNYRTKYPQGTITPKNPTAQSQVMNTDHKAYLDKNNAYPVECWIPDPSRNENTRYFGTYTGGENVPPVLHVTNTATTVLLDEQGVGPLCKADSLYVSAADICGLFTNSSGTQQWRGLARYFKIRLRKRSVKNPYPISFLLSDLINRRTQKVDGQPMYGMESQVEEVRVFDGTEQLPGDPDMIRYIDRQGQLQTKMV

SEQ ID NO: 3 - protein, 362 aa, Polyomavirus
MAPTKRKGECPGAAPKKPKEPVQVPKLLIKGGVEVLEVKTGVDAITEVECFLNPEMGDPDDHLRGYSQHLSAENAFDSDSPDKKMLPCYSTARIPLPNLNEDLTCGNLLMWEAVTVKTEVIGITSMLNLHAGSQKVHENGGGKPVQGSNFHFFAVGGDPLEMQGVLMNYRTKYPQGTITPKNPTAQSQVMNTDHKAYLDKNNAYPVECWIPDPSKNENTRYFGTYTGGENVPPVLHVTNTATTVLLDEQGVGPLCKADSLYVSAADICGLFTNSSGTQQWRGLARYFKIRLRKRSVKNPYPISFLLSDLINRRTQKVDGQPMYGMESQVEEVRVFDGTEQLPGDPDMIRYIDRQGQLQTKMV

SEQ ID NO: 4 - protein, 362 aa, Polyomavirus
MAPTKRKGECPGAAPKKPKEPVQVPKLLIKGGVEVLEVKTGVDAITEVECFLNPEMGDPDNDLRGYSLRLTAETAFDSDSPDRKMLPCYSTARIPLPNLNEDLTCGNLLMWEAVTVKTEVIGITSMLNLHAGSQKVHENGGGKPIQGSNFHFFAVGGDPLEMQGVLMNYRTKYPEGTVTPKNPTAQSQVMNTDHKAYLDKNNAYPVECWIPDPSRNENTRYFGTYTGGENVPPVLHVTNTATTVLLDEQGVGPLCKADSLYVSAADICGLFTNSSGTQQWRGLPRYFKIRLRKRSVKNPYPISFLLSDLINRRTQRVDGQPMYGMESQVEEVRVFDGTEQLPGDPDMIRYIDRQGQLQTKMV

SEQ ID NO: 5 - protein, 354 aa, Orthopolyomavirus
MAPTKRKGERKDPVQVPKLLIRGGVEVLEVKTGVDSITEVECFLTPEMGDPDEHLRGFSKSISISDTFESDSPNKDMLPCYSVARIPLPNLNEDLTCGNILMWEAVTLKTEVIGVTTLMNVHSNGQATHDNGAGKPVQGTSFHFFSVGGEALELQGVVFNYRTKYPDGTIFPKNATVQSQVMNTEHKAYLDKNKAYPVECWVPDPTRNENTRYFGTLTGGENVPPVLHITNTATTVLLDEFGVGPLCKGDNLYLSAVDVCGMFTNRSGSQQWRGLSRYFKVQLRKRRVKNPYPISFLLTDLINRRTPRVDGQPMYGMDAQVEEVRVFEGTEELPGDPDMMRYVDRYGQLQTKML

SEQ ID NO: 6 - protein, 5 aa, synthetic construct
  REGION 1..5: note = source = /note="Description of Artificial Sequence: Synthetic peptide"
NYWMT

SEQ ID NO: 7 - protein, 17 aa, synthetic construct
  REGION 1..17: note = source = /note="Description of Artificial Sequence: Synthetic peptide"
NIKKDGSEKYYVDSVRG

SEQ ID NO: 8 - protein, 11 aa, synthetic construct
  REGION 1..11: note = source = /note="Description of Artificial Sequence: Synthetic peptide"
VRSGRYFALDD

SEQ ID NO: 9 - protein, 7 aa, synthetic construct
  REGION 1..7: note = source = /note="Description of Artificial Sequence: Synthetic peptide"
GFTFNNY

SEQ ID NO: 10 - protein, 6 aa, synthetic construct
  REGION 1..6: note = source = /note="Description of Artificial Sequence: Synthetic peptide"
KKDGSE

SEQ ID NO: 11 - protein, 11 aa, synthetic construct
  REGION 1..11: note = source = /note="Description of Artificial Sequence: Synthetic peptide"
VRSGRYFALDD

SEQ ID NO: 12 - protein, 120 aa, synthetic construct
  REGION 1..120: note = source = /note="Description of Artificial Sequence: Synthetic polypeptide"
QVQLVESGGTLVQPGGSLRLSCAASGFTFNNYWMTWVRQAPGKGLEWVANIKKDGSEKYYVDSVRGRFTISRDNAKNSLFLQMNSLRPEDTAVYFCATVRSGRYFALDDWGQGTLVTVSS

SEQ ID NO: 13 - DNA, 360 bp, synthetic construct
  misc_feature 1..360: note = source = /note="Description of Artificial Sequence: Synthetic polynucleotide"
  source 1..360: mol_type = other DNA
caggtgcagctggtggaatcaggcggcacactggtgcagcctggcggtagcctgagactgagctgcgctgctagtggcttcacctttaacaactactggatgacctgggttaggcaggcccctggtaaaggcctcgagtgggtggcaaatatcaagaaggacggtagcgagaagtactacgtggactcagtcagaggccggttcactatctctagggataacgctaagaatagcctgttcctgcagatgaactcactgaggcccgaggataccgccgtctacttctgtgctaccgtcagatcaggccgctacttcgccctggacgactggggtcaaggcacactggtcaccgtgtctagc

SEQ ID NO: 14 - protein, 450 aa, synthetic construct
  REGION 1..450: note = source = /note="Description of Artificial Sequence: Synthetic polypeptide"
QVQLVESGGTLVQPGGSLRLSCAASGFTFNNYWMTWVRQAPGKGLEWVANIKKDGSEKYYVDSVRGRFTISRDNAKNSLFLQMNSLRPEDTAVYFCATVRSGRYFALDDWGQGTLVTVSSASTKGPSVFPLAPSSKSTSGGTAALGCLVKDYFPEPVTVSWNSGALTSGVHTFPAVLQSSGLYSLSSVVTVPSSSLGTQTYICNVNHKPSNTKVDKRVEPKSCDKTHTCPPCPAPELLGGPSVFLFPPKPKDTLMISRTPEVTCVVVDVSHEDPEVKFNWYVDGVEVHNAKTKPREEQYNSTYRVVSVLTVLHQDWLNGKEYKCKVSNKALPAPIEKTISKAKGQPREPQVYTLPPSREEMTKNQVSLTCLVKGFYPSDIAVEWESNGQPENNYKTTPPVLDSDGSFFLYSKLTVDKSRWQQGNVFSCSVMHEALHNHYTQKSLSLSPGK

SEQ ID NO: 15 - DNA, 1350 bp, synthetic construct
  misc_feature 1..1350: note = source = /note="Description of Artificial Sequence: Synthetic polynucleotide"
  source 1..1350: mol_type = other DNA
caggtgcagctggtggaatcaggcggcacactggtgcagcctggcggtagcctgagactgagctgcgctgctagtggcttcacctttaacaactactggatgacctgggttaggcaggcccctggtaaaggcctcgagtgggtggcaaatatcaagaaggacggtagcgagaagtactacgtggactcagtcagaggccggttcactatctctagggataacgctaagaatagcctgttcctgcagatgaactcactgaggcccgaggataccgccgtctacttctgtgctaccgtcagatcaggccgctacttcgccctggacgactggggtcaaggcacactggtcaccgtgtctagcgctagcactaagggcccaagtgtgtttcccctggcccccagcagcaagtctacttccggcggaactgctgccctgggttgcctggtgaaggactacttccccgagcccgtgacagtgtcctggaactctggggctctgacttccggcgtgcacaccttccccgccgtgctgcagagcagcggcctgtacagcctgagcagcgtggtgacagtgccctccagctctctgggaacccagacctatatctgcaacgtgaaccacaagcccagcaacaccaaggtggacaagagagtggagcccaagagctgcgacaagacccacacctgccccccctgcccagctccagaactgctgggagggccttccgtgttcctgttcccccccaagcccaaggacaccctgatgatcagcaggacccccgaggtgacctgcgtggtggtggacgtgtcccacgaggacccagaggtgaagttcaactggtacgtggacggcgtggaggtgcacaacgccaagaccaagcccagagaggagcagtacaacagcacctacagggtggtgtccgtgctgaccgtgctgcaccaggactggctgaacggcaaagaatacaagtgcaaagtctccaacaaggccctgccagccccaatcgaaaagacaatcagcaaggccaagggccagccacgggagccccaggtgtacaccctgccccccagccgggaggagatgaccaagaaccaggtgtccctgacctgtctggtgaagggcttctaccccagcgatatcgccgtggagtgggagagcaacggccagcccgagaacaactacaagaccacccccccagtgctggacagcgacggcagcttcttcctgtacagcaagctgaccgtggacaagtccaggtggcagcagggcaacgtgttcagctgcagcgtgatgcacgaggccctgcacaaccactacacccagaagtccctgagcctgagccccggcaag

SEQ ID NO: 16 - protein, 11 aa, synthetic construct
  REGION 1..11: note = source = /note="Description of Artificial Sequence: Synthetic peptide"
GGDNIGSRPVH

SEQ ID NO: 17 - protein, 7 aa, synthetic construct
  REGION 1..7: note = source = /note="Description of Artificial Sequence: Synthetic peptide"
DDSNRPS

SEQ ID NO: 18 - protein, 10 aa, synthetic construct
  REGION 1..10: note = source = /note="Description of Artificial Sequence: Synthetic peptide"
QVWSSSTDHP

SEQ ID NO: 19 - protein, 7 aa, synthetic construct
  REGION 1..7: note = source = /note="Description of Artificial Sequence: Synthetic peptide"
DNIGSRP

SEQ ID NO: 20 - skipped

SEQ ID NO: 21 - protein, 7 aa, synthetic construct
  REGION 1..7: note = source = /note="Description of Artificial Sequence: Synthetic peptide"
WSSSTDH

SEQ ID NO: 22 - protein, 107 aa, synthetic construct
  REGION 1..107: note = source = /note="Description of Artificial Sequence: Synthetic polypeptide"
QSVLTQPPSVSVAPGKTARITCGGDNIGSRPVHWYQQKPGQAPILVVYDDSNRPSGIPERFSGSNSGNTATLTISRVEAGDEADYYCQVWSSSTDHPFGGGTKVTVL

SEQ ID NO: 23 - DNA, 321 bp, synthetic construct
  misc_feature 1..321: note = source = /note="Description of Artificial Sequence: Synthetic polynucleotide"
  source 1..321: mol_type = other DNA
cagtcagtcctgactcagccccctagcgtcagcgtggcccctggtaaaaccgctagaatcacctgtggcggcgataatatcggctctaggcccgtgcactggtatcagcagaagcccggtcaagcccctatcctggtggtctacgacgactctaatagacctagcggaatccccgagcggtttagcggctctaattctggtaataccgctaccctgactatctctagggtggaagccggcgacgaggccgactactactgtcaagtctggtctagctctaccgatcaccccttcggcggaggcactaaggttacagtgctg

SEQ ID NO: 24 - protein, 213 aa, synthetic construct
  REGION 1..213: note = source = /note="Description of Artificial Sequence: Synthetic polypeptide"
QSVLTQPPSVSVAPGKTARITCGGDNIGSRPVHWYQQKPGQAPILVVYDDSNRPSGIPERFSGSNSGNTATLTISRVEAGDEADYYCQVWSSSTDHPFGGGTKVTVLGQPKAAPSVTLFPPSSEELQANKATLVCLISDFYPGAVTVAWKADSSPVKAGVETTTPSKQSNNKYAASSYLSLTPEQWKSHRSYSCQVTHEGSTVEKTVAPTECS

SEQ ID NO: 25 - DNA, 639 bp, synthetic construct
  misc_feature 1..639: note = source = /note="Description of Artificial Sequence: Synthetic polynucleotide"
  source 1..639: mol_type = other DNA
cagtcagtcctgactcagccccctagcgtcagcgtggcccctggtaaaaccgctagaatcacctgtggcggcgataatatcggctctaggcccgtgcactggtatcagcagaagcccggtcaagcccctatcctggtggtctacgacgactctaatagacctagcggaatccccgagcggtttagcggctctaattctggtaataccgctaccctgactatctctagggtggaagccggcgacgaggccgactactactgtcaagtctggtctagctctaccgatcaccccttcggcggaggcactaaggttacagtgctgggtcaacctaaggctgcccccagcgtgaccctgttcccccccagcagcgaggagctgcaggccaacaaggccaccctggtgtgcctgatcagcgacttctacccaggcgccgtgaccgtggcctggaaggccgacagcagccccgtgaaggccggcgtggagaccaccacccccagcaagcagagcaacaacaagtacgccgccagcagctacctgagcctgacccccgagcagtggaagagccacaggtcctacagctgccaggtgacccacgagggcagcaccgtggaaaagaccgtggccccaaccgagtgcagc

SEQ ID NO: 26 - protein, 5 aa, synthetic construct
  REGION 1..5: note = source = /note="Description of Artificial Sequence: Synthetic peptide"
NYWMT

SEQ ID NO: 27 - protein, 17 aa, synthetic construct
  REGION 1..17: note = source = /note="Description of Artificial Sequence: Synthetic peptide"
NIKKDGSEKYYVDSVRG

SEQ ID NO: 28 - protein, 11 aa, synthetic construct
  REGION 1..11: note = source = /note="Description of Artificial Sequence: Synthetic peptide"
VRSGRYFALDD

SEQ ID NO: 29 - protein, 7 aa, synthetic construct
  REGION 1..7: note = source = /note="Description of Artificial Sequence: Synthetic peptide"
GFTFSNY

SEQ ID NO: 30 - protein, 6 aa, synthetic construct
  REGION 1..6: note = source = /note="Description of Artificial Sequence: Synthetic peptide"
KKDGSE

SEQ ID NO: 31 - protein, 11 aa, synthetic construct
  REGION 1..11: note = source = /note="Description of Artificial Sequence: Synthetic peptide"
VRSGRYFALDD

SEQ ID NO: 32 - protein, 120 aa, synthetic construct
  REGION 1..120: note = source = /note="Description of Artificial Sequence: Synthetic polypeptide"
QVQLVESGGTLVQPGGSLRLSCAASGFTFSNYWMTWVRQAPGKGLEWVANIKKDGSEKYYVDSVRGRFTISRDNAKNSLFLQMNSLRPEDTAVYFCATVRSGRYFALDDWGQGTLVTVSS

SEQ ID NO: 33 - DNA, 360 bp, synthetic construct
  misc_feature 1..360: note = source = /note="Description of Artificial Sequence: Synthetic polynucleotide"
  source 1..360: mol_type = other DNA
caggtgcagctggtggaatcaggcggcacactggtgcagcctggcggtagcctgagactgagctgcgctgctagtggcttcaccttctctaactactggatgacctgggtcaggcaggcccctggtaaaggcctcgagtgggtggcaaatatcaagaaggacggtagcgagaagtactacgtggactcagtcagaggccggttcactatctctagggataacgctaagaatagcctgttcctgcagatgaactcactgaggcccgaggataccgccgtctacttctgtgctaccgtcagatcaggccgctacttcgccctggacgactggggtcaaggcacactggtcaccgtgtctagc

SEQ ID NO: 34 - protein, 450 aa, synthetic construct
  REGION 1..450: note = source = /note="Description of Artificial Sequence: Synthetic polypeptide"
QVQLVESGGTLVQPGGSLRLSCAASGFTFSNYWMTWVRQAPGKGLEWVANIKKDGSEKYYVDSVRGRFTISRDNAKNSLFLQMNSLRPEDTAVYFCATVRSGRYFALDDWGQGTLVTVSSASTKGPSVFPLAPSSKSTSGGTAALGCLVKDYFPEPVTVSWNSGALTSGVHTFPAVLQSSGLYSLSSVVTVPSSSLGTQTYICNVNHKPSNTKVDKRVEPKSCDKTHTCPPCPAPELLGGPSVFLFPPKPKDTLMISRTPEVTCVVVDVSHEDPEVKFNWYVDGVEVHNAKTKPREEQYNSTYRVVSVLTVLHQDWLNGKEYKCKVSNKALPAPIEKTISKAKGQPREPQVYTLPPSREEMTKNQVSLTCLVKGFYPSDIAVEWESNGQPENNYKTTPPVLDSDGSFFLYSKLTVDKSRWQQGNVFSCSVMHEALHNHYTQKSLSLSPGK

SEQ ID NO: 35 - DNA, 1350 bp, synthetic construct
  misc_feature 1..1350: note = source = /note="Description of Artificial Sequence: Synthetic polynucleotide"
  source 1..1350: mol_type = other DNA
caggtgcagctggtggaatcaggcggcacactggtgcagcctggcggtagcctgagactgagctgcgctgctagtggcttcaccttctctaactactggatgacctgggtcaggcaggcccctggtaaaggcctcgagtgggtggcaaatatcaagaaggacggtagcgagaagtactacgtggactcagtcagaggccggttcactatctctagggataacgctaagaatagcctgttcctgcagatgaactcactgaggcccgaggataccgccgtctacttctgtgctaccgtcagatcaggccgctacttcgccctggacgactggggtcaaggcacactggtcaccgtgtctagcgctagcactaagggcccaagtgtgtttcccctggcccccagcagcaagtctacttccggcggaactgctgccctgggttgcctggtgaaggactacttccccgagcccgtgacagtgtcctggaactctggggctctgacttccggcgtgcacaccttccccgccgtgctgcagagcagcggcctgtacagcctgagcagcgtggtgacagtgccctccagctctctgggaacccagacctatatctgcaacgtgaaccacaagcccagcaacaccaaggtggacaagagagtggagcccaagagctgcgacaagacccacacctgccccccctgcccagctccagaactgctgggagggccttccgtgttcctgttcccccccaagcccaaggacaccctgatgatcagcaggacccccgaggtgacctgcgtggtggtggacgtgtcccacgaggacccagaggtgaagttcaactggtacgtggacggcgtggaggtgcacaacgccaagaccaagcccagagaggagcagtacaacagcacctacagggtggtgtccgtgctgaccgtgctgcaccaggactggctgaacggcaaagaatacaagtgcaaagtctccaacaaggccctgccagccccaatcgaaaagacaatcagcaaggccaagggccagccacgggagccccaggtgtacaccctgccccccagccgggaggagatgaccaagaaccaggtgtccctgacctgtctggtgaagggcttctaccccagcgatatcgccgtggagtgggagagcaacggccagcccgagaacaactacaagaccacccccccagtgctggacagcgacggcagcttcttcctgtacagcaagctgaccgtggacaagtccaggtggcagcagggcaacgtgttcagctgcagcgtgatgcacgaggccctgcacaaccactacacccagaagtccctgagcctgagccccggcaag

SEQ ID NO: 36 - protein, 11 aa, synthetic construct
  REGION 1..11: note = source = /note="Description of Artificial Sequence: Synthetic peptide"
GGDNIGSRPVH

SEQ ID NO: 37 - protein, 7 aa, synthetic construct
  REGION 1..7: note = source = /note="Description of Artificial Sequence: Synthetic peptide"
DDSNRPS

SEQ ID NO: 38 - protein, 10 aa, synthetic construct
  REGION 1..10: note = source = /note="Description of Artificial Sequence: Synthetic peptide"
QVWSSSTDHP

SEQ ID NO: 39 - protein, 7 aa, synthetic construct
  REGION 1..7: note = source = /note="Description of Artificial Sequence: Synthetic peptide"
DNIGSRP

SEQ ID NO: 40 - skipped

SEQ ID NO: 41 - protein, 7 aa, synthetic construct
  REGION 1..7: note = source = /note="Description of Artificial Sequence: Synthetic peptide"
WSSSTDH

SEQ ID NO: 42 - protein, 107 aa, synthetic construct; identical to SEQ ID NO: 22
  REGION 1..107: note = source = /note="Description of Artificial Sequence: Synthetic polypeptide"

SEQ ID NO: 43 - DNA, 321 bp, synthetic construct; identical to SEQ ID NO: 23
  misc_feature 1..321: note = source = /note="Description of Artificial Sequence: Synthetic polynucleotide"
  source 1..321: mol_type = other DNA

SEQ ID NO: 44 - protein, 213 aa, synthetic construct; identical to SEQ ID NO: 24
  REGION 1..213: note = source = /note="Description of Artificial Sequence: Synthetic polypeptide"

SEQ ID NO: 45 - DNA, 639 bp, synthetic construct; identical to SEQ ID NO: 25
  misc_feature 1..639: note = source = /note="Description of Artificial Sequence: Synthetic polynucleotide"
  source 1..639: mol_type = other DNA

SEQ ID NO: 46 - protein, 5 aa, synthetic construct
  REGION 1..5: note = source = /note="Description of Artificial Sequence: Synthetic peptide"
NYWMT

SEQ ID NO: 47 - protein, 17 aa, synthetic construct
  REGION 1..17: note = source = /note="Description of Artificial Sequence: Synthetic peptide"
NIKKDGSEKYYVDSVRG

SEQ ID NO: 48 - protein, 11 aa, synthetic construct
  REGION 1..11: note = source = /note="Description of Artificial Sequence: Synthetic peptide"
VRSGRYFALDD

SEQ ID NO: 49 - protein, 7 aa, synthetic construct
  REGION 1..7: note = source = /note="Description of Artificial Sequence: Synthetic peptide"
GFTFKNY

SEQ ID NO: 50 - protein, 6 aa, synthetic construct
  REGION 1..6: note = source = /note="Description of Artificial Sequence: Synthetic peptide"
KKDGSE

SEQ ID NO: 51 - protein, 11 aa, synthetic construct
  REGION 1..11: note = source = /note="Description of Artificial Sequence: Synthetic peptide"
VRSGRYFALDD

SEQ ID NO: 52 - protein, 120 aa, synthetic construct
  REGION 1..120: note = source = /note="Description of Artificial Sequence: Synthetic polypeptide"
QVQLVESGGTLVQPGGSLRLSCAASGFTFKNYWMTWVRQAPGKGLEWVANIKKDGSEKYYVDSVRGRFTISRDNAKNSLFLQMNSLRPEDTAVYFCATVRSGRYFALDDWGQGTLVTVSS

SEQ ID NO: 53 - DNA, 360 bp, synthetic construct
  misc_feature 1..360: note = source = /note="Description of Artificial Sequence: Synthetic polynucleotide"
  source 1..360: mol_type = other DNA
caggtgcagctggtggaatcaggcggcacactggtgcagcctggcggtagcctgagactgagctgcgctgctagtggcttcacctttaagaactactggatgacctgggtcaggcaggcccctggtaaaggcctcgagtgggtggcaaatatcaagaaggacggtagcgagaagtactacgtggactcagtcagaggccggttcactatctctagggataacgctaagaatagcctgttcctgcagatgaactcactgaggcccgaggataccgccgtctacttctgtgctaccgtcagatcaggccgctacttcgccctggacgactggggtcaaggcacactggtcaccgtgtctagc

SEQ ID NO: 54 - protein, 450 aa, synthetic construct
  REGION 1..450: note = source = /note="Description of Artificial Sequence: Synthetic polypeptide"
QVQLVESGGTLVQPGGSLRLSCAASGFTFKNYWMTWVRQAPGKGLEWVANIKKDGSEKYYVDSVRGRFTISRDNAKNSLFLQMNSLRPEDTAVYFCATVRSGRYFALDDWGQGTLVTVSSASTKGPSVFPLAPSSKSTSGGTAALGCLVKDYFPEPVTVSWNSGALTSGVHTFPAVLQSSGLYSLSSVVTVPSSSLGTQTYICNVNHKPSNTKVDKRVEPKSCDKTHTCPPCPAPELLGGPSVFLFPPKPKDTLMISRTPEVTCVVVDVSHEDPEVKFNWYVDGVEVHNAKTKPREEQYNSTYRVVSVLTVLHQDWLNGKEYKCKVSNKALPAPIEKTISKAKGQPREPQVYTLPPSREEMTKNQVSLTCLVKGFYPSDIAVEWESNGQPENNYKTTPPVLDSDGSFFLYSKLTVDKSRWQQGNVFSCSVMHEALHNHYTQKSLSLSPGK

SEQ ID NO: 55 - DNA, 1350 bp, synthetic construct
  misc_feature 1..1350: note = source = /note="Description of Artificial Sequence: Synthetic polynucleotide"
  source 1..1350: mol_type = other DNA
caggtgcagctggtggaatcaggcggcacactggtgcagcctggcggtagcctgagactgagctgcgctgctagtggcttcacctttaagaactactggatgacctgggtcaggcaggcccctggtaaaggcctcgagtgggtggcaaatatcaagaaggacggtagcgagaagtactacgtggactcagtcagaggccggttcactatctctagggataacgctaagaatagcctgttcctgcagatgaactcactgaggcccgaggataccgccgtctacttctgtgctaccgtcagatcaggccgctacttcgccctggacgactggggtcaaggcacactggtcaccgtgtctagcgctagcactaagggcccaagtgtgtttcccctggcccccagcagcaagtctacttccggcggaactgctgccctgggttgcctggtgaaggactacttccccgagcccgtgacagtgtcctggaactctggggctctgacttccggcgtgcacaccttccccgccgtgctgcagagcagcggcctgtacagcctgagcagcgtggtgacagtgccctccagctctctgggaacccagacctatatctgcaacgtgaaccacaagcccagcaacaccaaggtggacaagagagtggagcccaagagctgcgacaagacccacacctgccccccctgcccagctccagaactgctgggagggccttccgtgttcctgttcccccccaagcccaaggacaccctgatgatcagcaggacccccgaggtgacctgcgtggtggtggacgtgtcccacgaggacccagaggtgaagttcaactggtacgtggacggcgtggaggtgcacaacgccaagaccaagcccagagaggagcagtacaacagcacctacagggtggtgtccgtgctgaccgtgctgcaccaggactggctgaacggcaaagaatacaagtgcaaagtctccaacaaggccctgccagccccaatcgaaaagacaatcagcaaggccaagggccagccacgggagccccaggtgtacaccctgccccccagccgggaggagatgaccaagaaccaggtgtccctgacctgtctggtgaagggcttctaccccagcgatatcgccgtggagtgggagagcaacggccagcccgagaacaactacaagaccacccccccagtgctggacagcgacggcagcttcttcctgtacagcaagctgaccgtggacaagtccaggtggcagcagggcaacgtgttcagctgcagcgtgatgcacgaggccctgcacaaccactacacccagaagtccctgagcctgagccccggcaag

SEQ ID NO: 56 - protein, 11 aa, synthetic construct
  REGION 1..11: note = source = /note="Description of Artificial Sequence: Synthetic peptide"
GGDNIGSRPVH

SEQ ID NO: 57 - protein, 7 aa, synthetic construct
  REGION 1..7: note = source = /note="Description of Artificial Sequence: Synthetic peptide"
DDSNRPS

SEQ ID NO: 58 - protein, 10 aa, synthetic construct
  REGION 1..10: note = source = /note="Description of Artificial Sequence: Synthetic peptide"
QVWSSSTDHP

SEQ ID NO: 59 - protein, 7 aa, synthetic construct
  REGION 1..7: note = source = /note="Description of Artificial Sequence: Synthetic peptide"
DNIGSRP

SEQ ID NO: 60 - skipped

SEQ ID NO: 61 - protein, 7 aa, synthetic construct
  REGION 1..7: note = source = /note="Description of Artificial Sequence: Synthetic peptide"
WSSSTDH

SEQ ID NO: 62 - protein, 107 aa, synthetic construct; identical to SEQ ID NO: 22
  REGION 1..107: note = source = /note="Description of Artificial Sequence: Synthetic polypeptide"

SEQ ID NO: 63 - DNA, 321 bp, synthetic construct; identical to SEQ ID NO: 23
  misc_feature 1..321: note = source = /note="Description of Artificial Sequence: Synthetic polynucleotide"
  source 1..321: mol_type = other DNA

SEQ ID NO: 64 - protein, 213 aa, synthetic construct; identical to SEQ ID NO: 24
  REGION 1..213: note = source = /note="Description of Artificial Sequence: Synthetic polypeptide"

SEQ ID NO: 65 - DNA, 639 bp, synthetic construct; identical to SEQ ID NO: 25
  misc_feature 1..639: note = source = /note="Description of Artificial Sequence: Synthetic polynucleotide"
  source 1..639: mol_type = other DNA

SEQ ID NO: 66 - protein, 5 aa, synthetic construct
  REGION 1..5: note = source = /note="Description of Artificial Sequence: Synthetic peptide"
NYWMT

SEQ ID NO: 67 - protein, 17 aa, synthetic construct
  REGION 1..17: note = source = /note="Description of Artificial Sequence: Synthetic peptide"
NIKKDGSEKYYVDSVRG

SEQ ID NO: 68 - protein, 11 aa, synthetic construct
  REGION 1..11: note = source = /note="Description of Artificial Sequence: Synthetic peptide"
VRSGRYFALDD

SEQ ID NO: 69 - protein, 7 aa, synthetic construct
  REGION 1..7: note = source = /note="Description of Artificial Sequence: Synthetic peptide"
GFTFQNY

SEQ ID NO: 70 - protein, 6 aa, synthetic construct
  REGION 1..6: note = source = /note="Description of Artificial Sequence: Synthetic peptide"
KKDGSE

SEQ ID NO: 71 - protein, 11 aa, synthetic construct
  REGION 1..11: note = source = /note="Description of Artificial Sequence: Synthetic peptide"
VRSGRYFALDD

SEQ ID NO: 72 - protein, 120 aa, synthetic construct
  REGION 1..120: note = source = /note="Description of Artificial Sequence: Synthetic polypeptide"
QVQLVESGGTLVQPGGSLRLSCAASGFTFQNYWMTWVRQAPGKGLEWVANIKKDGSEKYYVDSVRGRFTISRDNAKNSLFLQMNSLRPEDTAVYFCATVRSGRYFALDDWGQGTLVTVSS

SEQ ID NO: 73 - DNA, 360 bp, synthetic construct
  misc_feature 1..360: note = source = /note="Description of Artificial Sequence: Synthetic polynucleotide"
  source 1..360: mol_type = other DNA
caggtgcagctggtggaatcaggcggcacactggtgcagcctggcggtagcctgagactgagctgcgccgctagtggattcacctttcagaactactggatgacctgggtcagacaggcccctggtaaaggcctcgagtgggtggcaaatatcaagaaggacggtagcgagaagtactacgtggactcagtcagaggccggttcactatctctagggataacgctaagaatagcctgttcctgcagatgaactcactgaggcccgaggataccgccgtctacttctgtgctaccgtcagatcaggccgctacttcgccctggacgactggggtcaaggcacactggtcaccgtgtctagc

SEQ ID NO: 74 - protein, 450 aa, synthetic construct
  REGION 1..450: note = source = /note="Description of Artificial Sequence: Synthetic polypeptide"
QVQLVESGGTLVQPGGSLRLSCAASGFTFQNYWMTWVRQAPGKGLEWVANIKKDGSEKYYVDSVRGRFTISRDNAKNSLFLQMNSLRPEDTAVYFCATVRSGRYFALDDWGQGTLVTVSSASTKGPSVFPLAPSSKSTSGGTAALGCLVKDYFPEPVTVSWNSGALTSGVHTFPAVLQSSGLYSLSSVVTVPSSSLGTQTYICNVNHKPSNTKVDKRVEPKSCDKTHTCPPCPAPELLGGPSVFLFPPKPKDTLMISRTPEVTCVVVDVSHEDPEVKFNWYVDGVEVHNAKTKPREEQYNSTYRVVSVLTVLHQDWLNGKEYKCKVSNKALPAPIEKTISKAKGQPREPQVYTLPPSREEMTKNQVSLTCLVKGFYPSDIAVEWESNGQPENNYKTTPPVLDSDGSFFLYSKLTVDKSRWQQGNVFSCSVMHEALHNHYTQKSLSLSPGK

SEQ ID NO: 75 - DNA, 1350 bp, synthetic construct
  misc_feature 1..1350: note = source = /note="Description of Artificial Sequence: Synthetic polynucleotide"
  source 1..1350: mol_type = other DNA
caggtgcagctggtggaatcaggcggcacactggtgcagcctggcggtagcctgagactgagctgcgccgctagtggattcacctttcagaactactggatgacctgggtcagacaggcccctggtaaaggcctcgagtgggtggcaaatatcaagaaggacggtagcgagaagtactacgtggactcagtcagaggccggttcactatctctagggataacgctaagaatagcctgttcctgcagatgaactcactgaggcccgaggataccgccgtctacttctgtgctaccgtcagatcaggccgctacttcgccctggacgactggggtcaaggcacactggtcaccgtgtctagcgctagcactaagggcccaagtgtgtttcccctggcccccagcagcaagtctacttccggcggaactgctgccctgggttgcctggtgaaggactacttccccgagcccgtgacagtgtcctggaactctggggctctgacttccggcgtgcacaccttccccgccgtgctgcagagcagcggcctgtacagcctgagcagcgtggtgacagtgccctccagctctctgggaacccagacctatatctgcaacgtgaaccacaagcccagcaacaccaaggtggacaagagagtggagcccaagagctgcgacaagacccacacctgccccccctgcccagctccagaactgctgggagggccttccgtgttcctgttcccccccaagcccaaggacaccctgatgatcagcaggacccccgaggtgacctgcgtggtggtggacgtgtcccacgaggacccagaggtgaagttcaactggtacgtggacggcgtggaggtgcacaacgccaagaccaagcccagagaggagcagtacaacagcacctacagggtggtgtccgtgctgaccgtgctgcaccaggactggctgaacggcaaagaatacaagtgcaaagtctccaacaaggccctgccagccccaatcgaaaagacaatcagcaaggccaagggccagccacgggagccccaggtgtacaccctgccccccagccgggaggagatgaccaagaaccaggtgtccctgacctgtctggtgaagggcttctaccccagcgatatcgccgtggagtgggagagcaacggccagcccgagaacaactacaagaccacccccccagtgctggacagcgacggcagcttcttcctgtacagcaagctgaccgtggacaagtccaggtggcagcagggcaacgtgttcagctgcagcgtgatgcacgaggccctgcacaaccactacacccagaagtccctgagcctgagccccggcaag

SEQ ID NO: 76 - protein, 11 aa, synthetic construct
  REGION 1..11: note = source = /note="Description of Artificial Sequence: Synthetic peptide"
GGDNIGSRPVH

SEQ ID NO: 77 - protein, 7 aa, synthetic construct
  REGION 1..7: note = source = /note="Description of Artificial Sequence: Synthetic peptide"
DDSNRPS

SEQ ID NO: 78 - protein, 10 aa, synthetic construct
  REGION 1..10: note = source = /note="Description of Artificial Sequence: Synthetic peptide"
QVWSSSTDHP

SEQ ID NO: 79 - protein, 7 aa, synthetic construct
  REGION 1..7: note = source = /note="Description of Artificial Sequence: Synthetic peptide"
DNIGSRP

SEQ ID NO: 80-81 - skipped (2 entries)

SEQ ID NO: 82 - protein, 7 aa, synthetic construct
  REGION 1..7: note = source = /note="Description of Artificial Sequence: Synthetic peptide"
WSSSTDH

SEQ ID NO: 83 - protein, 107 aa, synthetic construct; identical to SEQ ID NO: 22
  REGION 1..107: note = source = /note="Description of Artificial Sequence: Synthetic polypeptide"

SEQ ID NO: 84 - DNA, 321 bp, synthetic construct; identical to SEQ ID NO: 23
  misc_feature 1..321: note = source = /note="Description of Artificial Sequence: Synthetic polynucleotide"
  source 1..321: mol_type = other DNA

SEQ ID NO: 85 - protein, 213 aa, synthetic construct; identical to SEQ ID NO: 24
  REGION 1..213: note = source = /note="Description of Artificial Sequence: Synthetic polypeptide"

SEQ ID NO: 86 - DNA, 639 bp, synthetic construct; identical to SEQ ID NO: 25
  misc_feature 1..639: note = source = /note="Description of Artificial Sequence: Synthetic polynucleotide"
  source 1..639: mol_type = other DNA

SEQ ID NO: 87 - protein, 5 aa, synthetic construct
  REGION 1..5: note = source = /note="Description of Artificial Sequence: Synthetic peptide"
NYWMT

SEQ ID NO: 88 - protein, 17 aa, synthetic construct
  REGION 1..17: note = source = /note="Description of Artificial Sequence: Synthetic peptide"
NIKKDGSEKYYVDSVRG

SEQ ID NO: 89 - protein, 11 aa, synthetic construct
  REGION 1..11: note = source = /note="Description of Artificial Sequence: Synthetic peptide"
VRSGRYFALDD

SEQ ID NO: 90 - protein, 7 aa, synthetic construct
  REGION 1..7: note = source = /note="Description of Artificial Sequence: Synthetic peptide"
GFTFNNY

SEQ ID NO: 91 - protein, 6 aa, synthetic construct
  REGION 1..6: note = source = /note="Description of Artificial Sequence: Synthetic peptide"
KKDGSE

SEQ ID NO: 92 - protein, 11 aa, synthetic construct
  REGION 1..11: note = source = /note="Description of Artificial Sequence: Synthetic peptide"
VRSGRYFALDD

SEQ ID NO: 93 - protein, 120 aa, synthetic construct
  REGION 1..120: note = source = /note="Description of Artificial Sequence: Synthetic polypeptide"
QVQLQESGPGLVQPGGSLRLSCAASGFTFNNYWMTWVRQAPGKGLEWVANIKKDGSEKYYVDSVRGRFTISRDNAKNSLFLQMNSLRPEDTAVYFCATVRSGRYFALDDWGQGTLVTVSS

SEQ ID NO: 94 - DNA, 360 bp, synthetic construct
  misc_feature 1..360: note = source = /note="Description of Artificial Sequence: Synthetic polynucleotide"
  source 1..360: mol_type = other DNA
caggtgcagctgcaggaatcaggcccaggactggtgcagcctggcggtagcctgagactgagctgcgctgctagtggcttcacctttaacaactactggatgacctgggtccgccaggcccctggcaaaggcctggagtgggtggcaaatatcaagaaggacggtagcgagaagtactacgtggactcagtcagaggccggttcactatctctagggataacgctaagaatagcctgttcctgcagatgaactcactgaggcccgaggataccgccgtctacttctgtgctaccgtcagatcaggccgctacttcgccctggacgactggggccagggcaccctggtcaccgtgtcttcc

SEQ ID NO: 95 - protein, 450 aa, synthetic construct
  REGION 1..450: note = source = /note="Description of Artificial Sequence: Synthetic polypeptide"
QVQLQESGPGLVQPGGSLRLSCAASGFTFNNYWMTWVRQAPGKGLEWVANIKKDGSEKYYVDSVRGRFTISRDNAKNSLFLQMNSLRPEDTAVYFCATVRSGRYFALDDWGQGTLVTVSSASTKGPSVFPLAPSSKSTSGGTAALGCLVKDYFPEPVTVSWNSGALTSGVHTFPAVLQSSGLYSLSSVVTVPSSSLGTQTYICNVNHKPSNTKVDKRVEPKSCDKTHTCPPCPAPELLGGPSVFLFPPKPKDTLMISRTPEVTCVVVDVSHEDPEVKFNWYVDGVEVHNAKTKPREEQYNSTYRVVSVLTVLHQDWLNGKEYKCKVSNKALPAPIEKTISKAKGQPREPQVYTLPPSREEMTKNQVSLTCLVKGFYPSDIAVEWESNGQPENNYKTTPPVLDSDGSFFLYSKLTVDKSRWQQGNVFSCSVMHEALHNHYTQKSLSLSPGK

SEQ ID NO: 96 - DNA, 1350 bp, synthetic construct
  misc_feature 1..1350: note = source = /note="Description of Artificial Sequence: Synthetic polynucleotide"
  source 1..1350: mol_type = other DNA
caggtgcagctgcaggaatcaggcccaggactggtgcagcctggcggtagcctgagactgagctgcgctgctagtggcttcacctttaacaactactggatgacctgggtccgccaggcccctggcaaaggcctggagtgggtggcaaatatcaagaaggacggtagcgagaagtactacgtggactcagtcagaggccggttcactatctctagggataacgctaagaatagcctgttcctgcagatgaactcactgaggcccgaggataccgccgtctacttctgtgctaccgtcagatcaggccgctacttcgccctggacgactggggccagggcaccctggtcaccgtgtcttccgctagcactaagggcccaagtgtgtttcccctggcccccagcagcaagtctacttccggcggaactgctgccctgggttgcctggtgaaggactacttccccgagcccgtgacagtgtcctggaactctggggctctgacttccggcgtgcacaccttccccgccgtgctgcagagcagcggcctgtacagcctgagcagcgtggtgacagtgccctccagctctctgggaacccagacctatatctgcaacgtgaaccacaagcccagcaacaccaaggtggacaagagagtggagcccaagagctgcgacaagacccacacctgccccccctgcccagctccagaactgctgggagggccttccgtgttcctgttcccccccaagcccaaggacaccctgatgatcagcaggacccccgaggtgacctgcgtggtggtggacgtgtcccacgaggacccagaggtgaagttcaactggtacgtggacggcgtggaggtgcacaacgccaagaccaagcccagagaggagcagtacaacagcacctacagggtggtgtccgtgctgaccgtgctgcaccaggactggctgaacggcaaagaatacaagtgcaaagtctccaacaaggccctgccagccccaatcgaaaagacaatcagcaaggccaagggccagccacgggagccccaggtgtacaccctgccccccagccgggaggagatgaccaagaaccaggtgtccctgacctgtctggtgaagggcttctaccccagcgatatcgccgtggagtgggagagcaacggccagcccgagaacaactacaagaccacccccccagtgctggacagcgacggcagcttcttcctgtacagcaagctgaccgtggacaagtccaggtggcagcagggcaacgtgttcagctgcagcgtgatgcacgaggccctgcacaaccactacacccagaagtccctgagcctgagccccggcaag

SEQ ID NO: 97 - protein, 11 aa, synthetic construct
  REGION 1..11: note = source = /note="Description of Artificial Sequence: Synthetic peptide"
GGDNIGSRPVH

SEQ ID NO: 98 - protein, 7 aa, synthetic construct
  REGION 1..7: note = source = /note="Description of Artificial Sequence: Synthetic peptide"
DDSNRPS

SEQ ID NO: 99 - protein, 10 aa, synthetic construct
  REGION 1..10: note = source = /note="Description of Artificial Sequence: Synthetic peptide"
QVWSSSTDHP

SEQ ID NO: 100 - protein, 7 aa, synthetic construct
  REGION 1..7: note = source = /note="Description of Artificial Sequence: Synthetic peptide"
DNIGSRP

SEQ ID NO: 101 - skipped

SEQ ID NO: 102 - protein, 7 aa, synthetic construct
  REGION 1..7: note = source = /note="Description of Artificial Sequence: Synthetic peptide"
WSSSTDH

SEQ ID NO: 103 - protein, 107 aa, synthetic construct; identical to SEQ ID NO: 22
  REGION 1..107: note = source = /note="Description of Artificial Sequence: Synthetic polypeptide"

SEQ ID NO: 104 - DNA, 321 bp, synthetic construct; identical to SEQ ID NO: 23
  misc_feature 1..321: note = source = /note="Description of Artificial Sequence: Synthetic polynucleotide"
  source 1..321: mol_type = other DNA

SEQ ID NO: 105 - protein, 213 aa, synthetic construct; identical to SEQ ID NO: 24
  REGION 1..213: note = source = /note="Description of Artificial Sequence: Synthetic polypeptide"

SEQ ID NO: 106 - DNA, 639 bp, synthetic construct; identical to SEQ ID NO: 25
  misc_feature 1..639: note = source = /note="Description of Artificial Sequence: Synthetic polynucleotide"
  source 1..639: mol_type = other DNA

SEQ ID NO: 107 - protein, 5 aa, synthetic construct
  REGION 1..5: note = source = /note="Description of Artificial Sequence: Synthetic peptide"
NYWMT

SEQ ID NO: 108 - protein, 17 aa, synthetic construct
  REGION 1..17: note = source = /note="Description of Artificial Sequence: Synthetic peptide"
NIKKDGSEKYYVDSVRG

SEQ ID NO: 109 - protein, 11 aa, synthetic construct
  REGION 1..11: note = source = /note="Description of Artificial Sequence: Synthetic peptide"
VRSGRYFALDD

SEQ ID NO: 110 - protein, 7 aa, synthetic construct
  REGION 1..7: note = source = /note="Description of Artificial Sequence: Synthetic peptide"
GFTFNNY

SEQ ID NO: 111 - protein, 6 aa, synthetic construct
  REGION 1..6: note = source = /note="Description of Artificial Sequence: Synthetic peptide"
KKDGSE

SEQ ID NO: 112 - protein, 11 aa, synthetic construct
  REGION 1..11: note = source = /note="Description of Artificial Sequence: Synthetic peptide"
VRSGRYFALDD

SEQ ID NO: 113 - protein, 120 aa, synthetic construct
  REGION 1..120: note = source = /note="Description of Artificial Sequence: Synthetic polypeptide"
QVQLVESGGGLVQPGGSLRLSCAASGFTFNNYWMTWVRQAPGKGLEWVANIKKDGSEKYYVDSVRGRFTISRDNAKNSLFLQMNSLRPEDTAVYFCATVRSGRYFALDDWGQGTLVTVSS

SEQ ID NO: 114 - DNA, 360 bp, synthetic construct
  misc_feature 1..360: note = source = /note="Description of Artificial Sequence: Synthetic polynucleotide"
  source 1..360: mol_type = other DNA
caggtgcagctggtggaatcaggcggcggactggtgcagcctggcggtagcctgagactgagctgcgctgctagtggcttcacctttaacaactactggatgacctgggttaggcaggcccctggtaaaggcctcgagtgggtggcaaatatcaagaaggacggtagcgagaagtactacgtggactcagtcagaggccggttcactatctctagggataacgctaagaatagcctgttcctgcagatgaactcactgaggcccgaggataccgccgtctacttctgtgctaccgtcagatcaggccgctacttcgccctggacgactggggtcaaggcacactggtcaccgtgtctagc

SEQ ID NO: 115 - protein, 450 aa, synthetic construct
  REGION 1..450: note = source = /note="Description of Artificial Sequence: Synthetic polypeptide"
QVQLVESGGGLVQPGGSLRLSCAASGFTFNNYWMTWVRQAPGKGLEWVANIKKDGSEKYYVDSVRGRFTISRDNAKNSLFLQMNSLRPEDTAVYFCATVRSGRYFALDDWGQGTLVTVSSASTKGPSVFPLAPSSKSTSGGTAALGCLVKDYFPEPVTVSWNSGALTSGVHTFPAVLQSSGLYSLSSVVTVPSSSLGTQTYICNVNHKPSNTKVDKRVEPKSCDKTHTCPPCPAPELLGGPSVFLFPPKPKDTLMISRTPEVTCVVVDVSHEDPEVKFNWYVDGVEVHNAKTKPREEQYNSTYRVVSVLTVLHQDWLNGKEYKCKVSNKALPAPIEKTISKAKGQPREPQVYTLPPSREEMTKNQVSLTCLVKGFYPSDIAVEWESNGQPENNYKTTPPVLDSDGSFFLYSKLTVDKSRWQQGNVFSCSVMHEALHNHYTQKSLSLSPGK

SEQ ID NO: 116 - DNA, 1350 bp, synthetic construct
  misc_feature 1..1350: note = source = /note="Description of Artificial Sequence: Synthetic polynucleotide"
  source 1..1350: mol_type = other DNA
caggtgcagctggtggaatcaggcggcggactggtgcagcctggcggtagcctgagactgagctgcgctgctagtggcttcacctttaacaactactggatgacctgggttaggcaggcccctggtaaaggcctcgagtgggtggcaaatatcaagaaggacggtagcgagaagtactacgtggactcagtcagaggccggttcactatctctagggataacgctaagaatagcctgttcctgcagatgaactcactgaggcccgaggataccgccgtctacttctgtgctaccgtcagatcaggccgctacttcgccctggacgactggggtcaaggcacactggtcaccgtgtctagcgctagcactaagggcccaagtgtgtttcccctggcccccagcagcaagtctacttccggcggaactgctgccctgggttgcctggtgaaggactacttccccgagcccgtgacagtgtcctggaactctggggctctgacttccggcgtgcacaccttccccgccgtgctgcagagcagcggcctgtacagcctgagcagcgtggtgacagtgccctccagctctctgggaacccagacctatatctgcaacgtgaaccacaagcccagcaacaccaaggtggacaagagagtggagcccaagagctgcgacaagacccacacctgccccccctgcccagctccagaactgctgggagggccttccgtgttcctgttcccccccaagcccaaggacaccctgatgatcagcaggacccccgaggtgacctgcgtggtggtggacgtgtcccacgaggacccagaggtgaagttcaactggtacgtggacggcgtggaggtgcacaacgccaagaccaagcccagagaggagcagtacaacagcacctacagggtggtgtccgtgctgaccgtgctgcaccaggactggctgaacggcaaagaatacaagtgcaaagtctccaacaaggccctgccagccccaatcgaaaagacaatcagcaaggccaagggccagccacgggagccccaggtgtacaccctgccccccagccgggaggagatgaccaagaaccaggtgtccctgacctgtctggtgaagggcttctaccccagcgatatcgccgtggagtgggagagcaacggccagcccgagaacaactacaagaccacccccccagtgctggacagcgacggcagcttcttcctgtacagcaagctgaccgtggacaagtccaggtggcagcagggcaacgtgttcagctgcagcgtgatgcacgaggccctgcacaaccactacacccagaagtccctgagcctgagccccggcaag

SEQ ID NO: 117 - protein, 11 aa, synthetic construct
  REGION 1..11: note = source = /note="Description of Artificial Sequence: Synthetic peptide"
GGDNIGSRPVH

SEQ ID NO: 118 - protein, 7 aa, synthetic construct
  REGION 1..7: note = source = /note="Description of Artificial Sequence: Synthetic peptide"
DDSNRPS

SEQ ID NO: 119 - protein, 10 aa, synthetic construct
  REGION 1..10: note = source = /note="Description of Artificial Sequence: Synthetic peptide"
QVWSSSTDHP

SEQ ID NO: 120 - protein, 7 aa, synthetic construct
  REGION 1..7: note = source = /note="Description of Artificial Sequence: Synthetic peptide"
DNIGSRP

SEQ ID NO: 121 - skipped

SEQ ID NO: 122 - protein, 7 aa, synthetic construct
  REGION 1..7: note = source = /note="Description of Artificial Sequence: Synthetic peptide"
WSSSTDH

SEQ ID NO: 123 - protein, 107 aa, synthetic construct; identical to SEQ ID NO: 22
  REGION 1..107: note = source = /note="Description of Artificial Sequence: Synthetic polypeptide"

SEQ ID NO: 124 - DNA, 321 bp, synthetic construct; identical to SEQ ID NO: 23
  misc_feature 1..321: note = source = /note="Description of Artificial Sequence: Synthetic polynucleotide"
  source 1..321: mol_type = other DNA

SEQ ID NO: 125 - protein, 213 aa, synthetic construct; identical to SEQ ID NO: 24
  REGION 1..213: note = source = /note="Description of Artificial Sequence: Synthetic polypeptide"

SEQ ID NO: 126 - DNA, 639 bp, synthetic construct; identical to SEQ ID NO: 25
  misc_feature 1..639: note = source = /note="Description of Artificial Sequence: Synthetic polynucleotide"
  source 1..639: mol_type = other DNA

SEQ ID NO: 127 - protein, 5 aa, synthetic construct
  REGION 1..5: note = source = /note="Description of Artificial Sequence: Synthetic peptide"
RDYWT

SEQ ID NO: 128 - protein, 16 aa, synthetic construct
  REGION 1..16: note = source = /note="Description of Artificial Sequence: Synthetic peptide"
NIYYSGSTNYNPSLKS

SEQ ID NO: 129 - protein, 16 aa, synthetic construct
  REGION 1..16: note = source = /note="Description of Artificial Sequence: Synthetic peptide"
VPGCSSTSCIDGWFDP

SEQ ID NO: 130 - protein, 7 aa, synthetic construct
  REGION 1..7: note = source = /note="Description of Artificial Sequence: Synthetic peptide"
GGSISRD

SEQ ID NO: 131 - protein, 5 aa, synthetic construct
  REGION 1..5: note = source = /note="Description of Artificial Sequence: Synthetic peptide"
YYSGS

SEQ ID NO: 132 - protein, 16 aa, synthetic construct
  REGION 1..16: note = source = /note="Description of Artificial Sequence: Synthetic peptide"
VPGCSSTSCIDGWFDP

SEQ ID NO: 133 - protein, 124 aa, synthetic construct
  REGION 1..124: note = source = /note="Description of Artificial Sequence: Synthetic polypeptide"
QVQLQESGPGLVKPSETLSLTCTVSGGSISRDYWTWVRQPPGEGLEWIGNIYYSGSTNYNPSLKSRVTISVAASKKQFSLKLTSVTAADTAVYYCARVPGCSSTSCIDGWFDPWGQGILVTVSS

SEQ ID NO: 134 - DNA, 372 bp, synthetic construct
  misc_feature 1..372: note = source = /note="Description of Artificial Sequence: Synthetic polynucleotide"
  source 1..372: mol_type = other DNA
caggtgcagctgcaagaatcaggccctggcctggtcaagcctagcgagacactgagcctgacctgcaccgtcagcggcggctctatctctagggactactggacctgggtccgacagcctcctggcgagggcctcgagtggatcggtaatatctactatagcggctctactaactataaccctagcctgaagtctagggtcacaattagcgtggccgcctctaagaagcagtttagcctgaagctgactagcgtgaccgccgctgacaccgccgtctactactgcgctagagtgcccggctgctctagcactagctgtatcgacggctggtttgacccttggggtcaagggatcctggtcaccgtgtctagc

SEQ ID NO: 135 - protein, 454 aa, synthetic construct
  REGION 1..454: note = source = /note="Description of Artificial Sequence: Synthetic polypeptide"
QVQLQESGPGLVKPSETLSLTCTVSGGSISRDYWTWVRQPPGEGLEWIGNIYYSGSTNYNPSLKSRVTISVAASKKQFSLKLTSVTAADTAVYYCARVPGCSSTSCIDGWFDPWGQGILVTVSSASTKGPSVFPLAPSSKSTSGGTAALGCLVKDYFPEPVTVSWNSGALTSGVHTFPAVLQSSGLYSLSSVVTVPSSSLGTQTYICNVNHKPSNTKVDKRVEPKSCDKTHTCPPCPAPELLGGPSVFLFPPKPKDTLMISRTPEVTCVVVDVSHEDPEVKFNWYVDGVEVHNAKTKPREEQYNSTYRVVSVLTVLHQDWLNGKEYKCKVSNKALPAPIEKTISKAKGQPREPQVYTLPPSREEMTKNQVSLTCLVKGFYPSDIAVEWESNGQPENNYKTTPPVLDSDGSFFLYSKLTVDKSRWQQGNVFSCSVMHEALHNHYTQKSLSLSPGK

SEQ ID NO: 136 - DNA, 1362 bp, synthetic construct
  misc_feature 1..1362: note = source = /note="Description of Artificial Sequence: Synthetic polynucleotide"
  source 1..1362: mol_type = other DNA
caggtgcagctgcaagaatcaggccctggcctggtcaagcctagcgagacactgagcctgacctgcaccgtcagcggcggctctatctctagggactactggacctgggtccgacagcctcctggcgagggcctcgagtggatcggtaatatctactatagcggctctactaactataaccctagcctgaagtctagggtcacaattagcgtggccgcctctaagaagcagtttagcctgaagctgactagcgtgaccgccgctgacaccgccgtctactactgcgctagagtgcccggctgctctagcactagctgtatcgacggctggtttgacccttggggtcaagggatcctggtcaccgtgtctagcgctagcactaagggcccaagtgtgtttcccctggcccccagcagcaagtctacttccggcggaactgctgccctgggttgcctggtgaaggactacttccccgagcccgtgacagtgtcctggaactctggggctctgacttccggcgtgcacaccttccccgccgtgctgcagagcagcggcctgtacagcctgagcagcgtggtgacagtgccctccagctctctgggaacccagacctatatctgcaacgtgaaccacaagcccagcaacaccaaggtggacaagagagtggagcccaagagctgcgacaagacccacacctgccccccctgcccagctccagaactgctgggagggccttccgtgttcctgttcccccccaagcccaaggacaccctgatgatcagcaggacccccgaggtgacctgcgtggtggtggacgtgtcccacgaggacccagaggtgaagttcaactggtacgtggacggcgtggaggtgcacaacgccaagaccaagcccagagaggagcagtacaacagcacctacagggtggtgtccgtgctgaccgtgctgcaccaggactggctgaacggcaaagaatacaagtgcaaagtctccaacaaggccctgccagccccaatcgaaaagacaatcagcaaggccaagggccagccacgggagccccaggtgtacaccctgccccccagccgggaggagatgaccaagaaccaggtgtccctgacctgtctggtgaagggcttctaccccagcgatatcgccgtggagtgggagagcaacggccagcccgagaacaactacaagaccacccccccagtgctggacagcgacggcagcttcttcctgtacagcaagctgaccgtggacaagtccaggtggcagcagggcaacgtgttcagctgcagcgtgatgcacgaggccctgcacaaccactacacccagaagtccctgagcctgagccccggcaag

SEQ ID NO: 137 - protein, 13 aa, synthetic construct
  REGION 1..13: note = source = /note="Description of Artificial Sequence: Synthetic peptide"
SGSSSNIGNTYVS

SEQ ID NO: 138 - protein, 7 aa, synthetic construct
  REGION 1..7: note = source = /note="Description of Artificial Sequence: Synthetic peptide"
DNNKRPS

SEQ ID NO: 139 - protein, 11 aa, synthetic construct
  REGION 1..11: note = source = /note="Description of Artificial Sequence: Synthetic peptide"
GTWDSSLSAWV

SEQ ID NO: 140 - protein, 9 aa, synthetic construct
  REGION 1..9: note = source = /note="Description of Artificial Sequence: Synthetic peptide"
SSSNIGNTY

SEQ ID NO: 141 - skipped

SEQ ID NO: 142 - protein, 8 aa, synthetic construct
  REGION 1..8: note = source = /note="Description of Artificial Sequence: Synthetic peptide"
WDSSLSAW

SEQ ID NO: 143 - protein, 110 aa, synthetic construct
  REGION 1..110: note = source = /note="Description of Artificial Sequence: Synthetic polypeptide"
QSVLTQPPSLSAAPGQRVTISCSGSSSNIGNTYVSWYQQLPGTAPKLLIYDNNKRPSGIPGRFSGSKSGTSATLGITGLQTGDEAAYYCGTWDSSLSAWVFGGGTRLTVL

SEQ ID NO: 144 - DNA, 330 bp, synthetic construct
  misc_feature 1..330: note = source = /note="Description of Artificial Sequence: Synthetic polynucleotide"
  source 1..330: mol_type = other DNA
cagtcagtcctgactcagccccctagcctgagcgccgctcccggtcaaagagtgactattagctgtagcggctctagctctaatatcggtaatacctacgtcagctggtatcagcagctgcccggcaccgcccctaagctgctgatctacgataacaacaagcggcctagcggaatccctggtcgctttagcggatctaaatcaggcactagcgctaccctgggaatcaccggcctgcagaccggcgacgaagccgcctactactgcggcacctgggactctagtctgagcgcctgggtgttcggcggaggcactagactgaccgtgctg

SEQ ID NO: 145 - protein, 216 aa, synthetic construct
  REGION 1..216: note = source = /note="Description of Artificial Sequence: Synthetic polypeptide"
QSVLTQPPSLSAAPGQRVTISCSGSSSNIGNTYVSWYQQLPGTAPKLLIYDNNKRPSGIPGRFSGSKSGTSATLGITGLQTGDEAAYYCGTWDSSLSAWVFGGGTRLTVLGQPKAAPSVTLFPPSSEELQANKATLVCLISDFYPGAVTVAWKADSSPVKAGVETTTPSKQSNNKYAASSYLSLTPEQWKSHRSYSCQVTHEGSTVEKTVAPTECS

SEQ ID NO: 146 - DNA, 648 bp, synthetic construct
  misc_feature 1..648: note = source = /note="Description of Artificial Sequence: Synthetic polynucleotide"
  source 1..648: mol_type = other DNA
cagtcagtcctgactcagccccctagcctgagcgccgctcccggtcaaagagtgactattagctgtagcggctctagctctaatatcggtaatacctacgtcagctggtatcagcagctgcccggcaccgcccctaagctgctgatctacgataacaacaagcggcctagcggaatccctggtcgctttagcggatctaaatcaggcactagcgctaccctgggaatcaccggcctgcagaccggcgacgaagccgcctactactgcggcacctgggactctagtctgagcgcctgggtgttcggcggaggcactagactgaccgtgctgggtcaacctaaggctgcccccagcgtgaccctgttcccccccagcagcgaggagctgcaggccaacaaggccaccctggtgtgcctgatcagcgacttctacccaggcgccgtgaccgtggcctggaaggccgacagcagccccgtgaaggccggcgtggagaccaccacccccagcaagcagagcaacaacaagtacgccgccagcagctacctgagcctgacccccgagcagtggaagagccacaggtcctacagctgccaggtgacccacgagggcagcaccgtggaaaagaccgtggccccaaccgagtgcagc

SEQ ID NO: 147 - protein, 5 aa, synthetic construct
  REGION 1..5: note = source = /note="Description of Artificial Sequence: Synthetic peptide"
RDYWS

SEQ ID NO: 148 - protein, 16 aa, synthetic construct
  REGION 1..16: note = source = /note="Description of Artificial Sequence: Synthetic peptide"
NIYYSGSTNYNPSLKS

SEQ ID NO: 149 - protein, 16 aa, synthetic construct
  REGION 1..16: note = source = /note="Description of Artificial Sequence: Synthetic peptide"
VPGCSSTSCIDGWFDP

SEQ ID NO: 150 - protein, 7 aa, synthetic construct
  REGION 1..7: note = source = /note="Description of Artificial Sequence: Synthetic peptide"
GGSISRD

SEQ ID NO: 151 - protein, 5 aa, synthetic construct
  REGION 1..5: note = source = /note="Description of Artificial Sequence: Synthetic peptide"
YYSGS

SEQ ID NO: 152 - protein, 16 aa, synthetic construct
  REGION 1..16: note = source = /note="Description of Artificial Sequence: Synthetic peptide"
VPGCSSTSCIDGWFDP

SEQ ID NO: 153 - protein, 124 aa, synthetic construct
  REGION 1..124: note = source = /note="Description of Artificial Sequence: Synthetic polypeptide"
QVQLQESGPGLVKPSETLSLTCTVSGGSISRDYWSWVRQPPGAGLEWIGNIYYSGSTNYNPSLKSRVTISVATNKKQFSLKLTSVTAADTAVYYCARVPGCSSTSCIDGWFDPWGQGILVTVSS

SEQ ID NO: 154 - DNA, 372 bp, synthetic construct
  misc_feature 1..372: note = source = /note="Description of Artificial Sequence: Synthetic polynucleotide"
  source 1..372: mol_type = other DNA
caggtgcagctgcaagaatcaggccctggcctggtcaagcctagcgagacactgagcctgacctgcaccgtcagcggcggctctatctctagggactactggtcctgggtccgacaacctcctggcgctggcctcgagtggatcggtaatatctactatagcggctctactaactataaccctagcctgaagtctagggtcacaattagtgtggctactaacaagaagcagtttagcctgaagctgactagcgtgaccgccgctgacaccgccgtctactactgcgctagagtgcccggctgctctagcactagctgtatcgacggttggtttgacccttggggtcaagggatcctggtcaccgtgtctagc

SEQ ID NO: 155 - protein, 454 aa, synthetic construct
  REGION 1..454: note = source = /note="Description of Artificial Sequence: Synthetic polypeptide"
QVQLQESGPGLVKPSETLSLTCTVSGGSISRDYWSWVRQPPGAGLEWIGNIYYSGSTNYNPSLKSRVTISVATNKKQFSLKLTSVTAADTAVYYCARVPGCSSTSCIDGWFDPWGQGILVTVSSASTKGPSVFPLAPSSKSTSGGTAALGCLVKDYFPEPVTVSWNSGALTSGVHTFPAVLQSSGLYSLSSVVTVPSSSLGTQTYICNVNHKPSNTKVDKRVEPKSCDKTHTCPPCPAPELLGGPSVFLFPPKPKDTLMISRTPEVTCVVVDVSHEDPEVKFNWYVDGVEVHNAKTKPREEQYNSTYRVVSVLTVLHQDWLNGKEYKCKVSNKALPAPIEKTISKAKGQPREPQVYTLPPSREEMTKNQVSLTCLVKGFYPSDIAVEWESNGQPENNYKTTPPVLDSDGSFFLYSKLTVDKSRWQQGNVFSCSVMHEALHNHYTQKSLSLSPGK

SEQ ID NO: 156 - DNA, 1362 bp, synthetic construct
  misc_feature 1..1362: note = source = /note="Description of Artificial Sequence: Synthetic polynucleotide"
  source 1..1362: mol_type = other DNA
caggtgcagctgcaagaatcaggccctggcctggtcaagcctagcgagacactgagcctgacctgcaccgtcagcggcggctctatctctagggactactggtcctgggtccgacaacctcctggcgctggcctcgagtggatcggtaatatctactatagcggctctactaactataaccctagcctgaagtctagggtcacaattagtgtggctactaacaagaagcagtttagcctgaagctgactagcgtgaccgccgctgacaccgccgtctactactgcgctagagtgcccggctgctctagcactagctgtatcgacggttggtttgacccttggggtcaagggatcctggtcaccgtgtctagcgctagcactaagggcccaagtgtgtttcccctggcccccagcagcaagtctacttccggcggaactgctgccctgggttgcctggtgaaggactacttccccgagcccgtgacagtgtcctggaactctggggctctgacttccggcgtgcacaccttccccgccgtgctgcagagcagcggcctgtacagcctgagcagcgtggtgacagtgccctccagctctctgggaacccagacctatatctgcaacgtgaaccacaagcccagcaacaccaaggtggacaagagagtggagcccaagagctgcgacaagacccacacctgccccccctgcccagctccagaactgctgggagggccttccgtgttcctgttcccccccaagcccaaggacaccctgatgatcagcaggacccccgaggtgacctgcgtggtggtggacgtgtcccacgaggacccagaggtgaagttcaactggtacgtggacggcgtggaggtgcacaacgccaagaccaagcccagagaggagcagtacaacagcacctacagggtggtgtccgtgctgaccgtgctgcaccaggactggctgaacggcaaagaatacaagtgcaaagtctccaacaaggccctgccagccccaatcgaaaagacaatcagcaaggccaagggccagccacgggagccccaggtgtacaccctgccccccagccgggaggagatgaccaagaaccaggtgtccctgacctgtctggtgaagggcttctaccccagcgatatcgccgtggagtgggagagcaacggccagcccgagaacaactacaagaccacccccccagtgctggacagcgacggcagcttcttcctgtacagcaagctgaccgtggacaagtccaggtggcagcagggcaacgtgttcagctgcagcgtgatgcacgaggccctgcacaaccactacacccagaagtccctgagcctgagccccggcaag

SEQ ID NO: 157 - protein, 13 aa, synthetic construct
  REGION 1..13: note = source = /note="Description of Artificial Sequence: Synthetic peptide"
SGSSSNIGNTYVS

SEQ ID NO: 158 - protein, 7 aa, synthetic construct
  REGION 1..7: note = source = /note="Description of Artificial Sequence: Synthetic peptide"
DNNKRPS

SEQ ID NO: 159 - protein, 11 aa, synthetic construct
  REGION 1..11: note = source = /note="Description of Artificial Sequence: Synthetic peptide"
GTWDSSLSAWV

SEQ ID NO: 160 - protein, 9 aa, synthetic construct
  REGION 1..9: note = source = /note="Description of Artificial Sequence: Synthetic peptide"
SSSNIGNTY

SEQ ID NO: 161 - skipped

SEQ ID NO: 162 - protein, 8 aa, synthetic construct
  REGION 1..8: note = source = /note="Description of Artificial Sequence: Synthetic peptide"
WDSSLSAW

SEQ ID NO: 163 - protein, 110 aa, synthetic construct
  REGION 1..110: note = source = /note="Description of Artificial Sequence: Synthetic polypeptide"
QSVLTQPPSLSAAPGQKVTISCSGSSSNIGNTYVSWYQQLPGTAPKLLIYDNNKRPSGIPDRFSGSKSGTSATLGITGLQTGDEAVYYCGTWDSSLSAWVFGGGTRLTVL

SEQ ID NO: 164 - DNA, 330 bp, synthetic construct
  misc_feature 1..330: note = source = /note="Description of Artificial Sequence: Synthetic polynucleotide"
  source 1..330: mol_type = other DNA
cagtcagtcctgactcagccccctagcctgagcgccgctcccggtcaaaaagtgactattagctgtagcggctctagctctaatatcggtaatacctacgtcagctggtatcagcagctgcccggcaccgcccctaagctgctgatctacgataacaacaagcggcctagcggaatccccgataggtttagcggatctaagtcaggcactagcgctaccctgggaatcaccggcctgcagaccggcgacgaggccgtctactactgcggcacctgggactctagtctgagcgcctgggtgttcggcggaggcactagactgaccgtgctg

SEQ ID NO: 165 - protein, 216 aa, synthetic construct
  REGION 1..216: note = source = /note="Description of Artificial Sequence: Synthetic polypeptide"
QSVLTQPPSLSAAPGQKVTISCSGSSSNIGNTYVSWYQQLPGTAPKLLIYDNNKRPSGIPDRFSGSKSGTSATLGITGLQTGDEAVYYCGTWDSSLSAWVFGGGTRLTVLGQPKAAPSVTLFPPSSEELQANKATLVCLISDFYPGAVTVAWKADSSPVKAGVETTTPSKQSNNKYAASSYLSLTPEQWKSHRSYSCQVTHEGSTVEKTVAPTECS

SEQ ID NO: 166 - DNA, 648 bp, synthetic construct
  misc_feature 1..648: note = source = /note="Description of Artificial Sequence: Synthetic polynucleotide"
  source 1..648: mol_type = other DNA
cagtcagtcctgactcagccccctagcctgagcgccgctcccggtcaaaaagtgactattagctgtagcggctctagctctaatatcggtaatacctacgtcagctggtatcagcagctgcccggcaccgcccctaagctgctgatctacgataacaacaagcggcctagcggaatccccgataggtttagcggatctaagtcaggcactagcgctaccctgggaatcaccggcctgcagaccggcgacgaggccgtctactactgcggcacctgggactctagtctgagcgcctgggtgttcggcggaggcactagactgaccgtgctgggtcaacctaaggctgcccccagcgtgaccctgttcccccccagcagcgaggagctgcaggccaacaaggccaccctggtgtgcctgatcagcgacttctacccaggcgccgtgaccgtggcctggaaggccgacagcagccccgtgaaggccggcgtggagaccaccacccccagcaagcagagcaacaacaagtacgccgccagcagctacctgagcctgacccccgagcagtggaagagccacaggtcctacagctgccaggtgacccacgagggcagcaccgtggaaaagaccgtggccccaaccgagtgcagc

SEQ ID NO: 167 - protein, 5 aa, synthetic construct
  REGION 1..5: note = source = /note="Description of Artificial Sequence: Synthetic peptide"
RDYWS

SEQ ID NO: 168 - protein, 16 aa, synthetic construct
  REGION 1..16: note = source = /note="Description of Artificial Sequence: Synthetic peptide"
NIYYSGSTNYNPSLKS

SEQ ID NO: 169 - protein, 16 aa, synthetic construct
  REGION 1..16: note = source = /note="Description of Artificial Sequence: Synthetic peptide"
VPGCSSTSCIDGWFDP

SEQ ID NO: 170 - protein, 7 aa, synthetic construct
  REGION 1..7: note = source = /note="Description of Artificial Sequence: Synthetic peptide"
GGSISRD

SEQ ID NO: 171 - protein, 5 aa, synthetic construct
  REGION 1..5: note = source = /note="Description of Artificial Sequence: Synthetic peptide"
YYSGS

SEQ ID NO: 172 - protein, 16 aa, synthetic construct
  REGION 1..16: note = source = /note="Description of Artificial Sequence: Synthetic peptide"
VPGCSSTSCIDGWFDP

SEQ ID NO: 173 - protein, 124 aa, synthetic construct; identical to SEQ ID NO: 153
  REGION 1..124: note = source = /note="Description of Artificial Sequence: Synthetic polypeptide"

SEQ ID NO: 174 - DNA, 372 bp, synthetic construct
  misc_feature 1..372: note = source = /note="Description of Artificial Sequence: Synthetic polynucleotide"
  source 1..372: mol_type = other DNA
caggtgcaattgcaggaaagcggccctggcctcgtgaagcccagcgagacactgagcctgacctgtaccgtgtccggcggcagcatcagcagagactactggagctgggttcgccagcctccaggcgcaggactggaatggatcggcaacatctactacagcggcagcaccaactacaaccccagcctgaagtccagagtgaccatcagcgtggccacaaacaagaaacagttctccctgaagctgaccagcgtgacagccgccgataccgccgtgtactactgcgccagagtgcctggctgtagcagcaccagctgcatcgacggatggttcgacccttggggccagggcattctcgtgaccgtcagctca

SEQ ID NO: 175 - protein, 454 aa, synthetic construct; identical to SEQ ID NO: 155
  REGION 1..454: note = source = /note="Description of Artificial Sequence: Synthetic polypeptide"

SEQ ID NO: 176 - DNA, 1362 bp, synthetic construct
  misc_feature 1..1362: note = source = /note="Description of Artificial Sequence: Synthetic polynucleotide"
  source 1..1362: mol_type = other DNA
caggtgcaattgcaggaaagcggccctggcctcgtgaagcccagcgagacactgagcctgacctgtaccgtgtccggcggcagcatcagcagagactactggagctgggttcgccagcctccaggcgcaggactggaatggatcggcaacatctactacagcggcagcaccaactacaaccccagcctgaagtccagagtgaccatcagcgtggccacaaacaagaaacagttctccctgaagctgaccagcgtgacagccgccgataccgccgtgtactactgcgccagagtgcctggctgtagcagcaccagctgcatcgacggatggttcgacccttggggccagggcattctcgtgaccgtcagctcagctagcaccaagggccccagcgtgttccccctggcccccagcagcaagagcaccagcggcggcacagccgccctgggctgcctggtgaaggactacttccccgagcccgtgaccgtgtcctggaacagcggagccctgacctccggcgtgcacaccttccccgccgtgctgcagagcagcggcctgtacagcctgtccagcgtggtgacagtgcccagcagcagcctgggcacccagacctacatctgcaacgtgaaccacaagcccagcaacaccaaggtggacaagagagtggagcccaagagctgcgacaagacccacacctgccccccctgcccagccccagagctgctgggcggaccctccgtgttcctgttcccccccaagcccaaggacaccctgatgatcagcaggacccccgaggtgacctgcgtggtggtggacgtgagccacgaggacccagaggtgaagttcaactggtacgtggacggcgtggaggtgcacaacgccaagaccaagcccagagaggagcagtacaacagcacctacagggtggtgtccgtgctgaccgtgctgcaccaggactggctgaacggcaaggaatacaagtgcaaggtctccaacaaggccctgccagcccccatcgaaaagaccatcagcaaggccaagggccagccacgggagccccaggtgtacaccctgcccccctcccgggaggagatgaccaagaaccaggtgtccctgacctgtctggtgaagggcttctaccccagcgacatcgccgtggagtgggagagcaacggccagcccgagaacaactacaagaccacccccccagtgctggacagcgacggcagcttcttcctgtacagcaagctgaccgtggacaagtccaggtggcagcagggcaacgtgttcagctgcagcgtgatgcacgaggccctgcacaaccactacacccagaagagcctgagcctgtcccccggcaag

SEQ ID NO: 177 - protein, 13 aa, synthetic construct
  REGION 1..13: note = source = /note="Description of Artificial Sequence: Synthetic peptide"
SGSSSNIGNTYVS

SEQ ID NO: 178 - protein, 7 aa, synthetic construct
  REGION 1..7: note = source = /note="Description of Artificial Sequence: Synthetic peptide"
DNNKRPS

SEQ ID NO: 179 - protein, 11 aa, synthetic construct
  REGION 1..11: note = source = /note="Description of Artificial Sequence: Synthetic peptide"
GTWDSSLSAWV

SEQ ID NO: 180 - protein, 9 aa, synthetic construct
  REGION 1..9: note = source = /note="Description of Artificial Sequence: Synthetic peptide"
SSSNIGNTY

SEQ ID NO: 181 - skipped

SEQ ID NO: 182 - protein, 8 aa, synthetic construct
  REGION 1..8: note = source = /note="Description of Artificial Sequence: Synthetic peptide"
WDSSLSAW

SEQ ID NO: 183 - protein, 110 aa, synthetic construct
  REGION 1..110: note = source = /note="Description of Artificial Sequence: Synthetic polypeptide"
QSVLTQPPSVSAAPGQKVTISCSGSSSNIGNTYVSWYQQLPGTAPKLLIYDNNKRPSGIPDRFSGSKSGTSATLGITGLQTGDEADYYCGTWDSSLSAWVFGGGTRLTVL

SEQ ID NO: 184 - DNA, 330 bp, synthetic construct
  misc_feature 1..330: note = source = /note="Description of Artificial Sequence: Synthetic polynucleotide"
  source 1..330: mol_type = other DNA
caaagcgtgctgacccagcctcctagcgtgtctgctgcccctggccagaaggtgaccatcagctgtagcggcagcagctccaacatcggcaacacctacgtgtcctggtatcagcagctgcccggcaccgcccccaaactgctgatctacgacaacaacaagcggcccagcggcatccccgatagattttctggcagcaagagcggcaccagcgccaccctgggaatcacaggactgcagacaggggacgaggccgattactactgtggcacctgggattctagcctgagcgcctgggtgttcggcggaggcacaagactgacagtgctg

SEQ ID NO: 185 - protein, 216 aa, synthetic construct
  REGION 1..216: note = source = /note="Description of Artificial Sequence: Synthetic polypeptide"
QSVLTQPPSVSAAPGQKVTISCSGSSSNIGNTYVSWYQQLPGTAPKLLIYDNNKRPSGIPDRFSGSKSGTSATLGITGLQTGDEADYYCGTWDSSLSAWVFGGGTRLTVLGQPKAAPSVTLFPPSSEELQANKATLVCLISDFYPGAVTVAWKADSSPVKAGVETTTPSKQSNNKYAASSYLSLTPEQWKSHRSYSCQVTHEGSTVEKTVAPTECS

SEQ ID NO: 186 - DNA, 648 bp, synthetic construct
  misc_feature 1..648: note = source = /note="Description of Artificial Sequence: Synthetic polynucleotide"
  source 1..648: mol_type = other DNA
caaagcgtgctgacccagcctcctagcgtgtctgctgcccctggccagaaggtgaccatcagctgtagcggcagcagctccaacatcggcaacacctacgtgtcctggtatcagcagctgcccggcaccgcccccaaactgctgatctacgacaacaacaagcggcccagcggcatccccgatagattttctggcagcaagagcggcaccagcgccaccctgggaatcacaggactgcagacaggggacgaggccgattactactgtggcacctgggattctagcctgagcgcctgggtgttcggcggaggcacaagactgacagtgctgggtcagcctaaggccgctccctccgtgaccctgttcccccccagctccgaggaactgcaggccaacaaggccaccctggtgtgcctgatcagcgacttctaccctggcgccgtgaccgtggcctggaaggccgacagcagccccgtgaaggccggcgtggagacaaccacccccagcaagcagagcaacaacaagtacgccgccagcagctacctgagcctgacccccgagcagtggaagagccacagaagctacagctgccaggtcacccacgagggcagcaccgtggagaaaaccgtggcccccaccgagtgcagc

SEQ ID NO: 187 - protein, 7 aa, synthetic construct
  REGION 1..7: note = source = /note="Description of Artificial Sequence: Synthetic peptide"
SGGYSWS

SEQ ID NO: 188 - protein, 16 aa, synthetic construct
  REGION 1..16: note = source = /note="Description of Artificial Sequence: Synthetic peptide"
YIYYRGTTYYNPSLKS

SEQ ID NO: 189 - protein, 13 aa, synthetic construct
  REGION 1..13: note = source = /note="Description of Artificial Sequence: Synthetic peptide"
ALTHLVGVGWFDP

SEQ ID NO: 190 - protein, 9 aa, synthetic construct
  REGION 1..9: note = source = /note="Description of Artificial Sequence: Synthetic peptide"
GGSISSGGY

SEQ ID NO: 191 - protein, 5 aa, synthetic construct
  REGION 1..5: note = source = /note="Description of Artificial Sequence: Synthetic peptide"
YYRGT

SEQ ID NO: 192 - protein, 13 aa, synthetic construct
  REGION 1..13: note = source = /note="Description of Artificial Sequence: Synthetic peptide"
ALTHLVGVGWFDP

SEQ ID NO: 193 - protein, 123 aa, synthetic construct
  REGION 1..123: note = source = /note="Description of Artificial Sequence: Synthetic polypeptide"
QVQLQESGPGLAKPSQTLSLTCSVSGGSISSGGYSWSWIRQPPGKGLEYIGYIYYRGTTYYNPSLKSRITMSVDTSNNQISLKLTSVTAADTAVYYCARALTHLVGVGWFDPWGQGTMVTVSS

SEQ ID NO: 194 - DNA, 369 bp, synthetic construct
  misc_feature 1..369: note = source = /note="Description of Artificial Sequence: Synthetic polynucleotide"
  source 1..369: mol_type = other DNA
caggtgcagctgcaagaatcaggccctggcctggctaagcctagtcagaccctgagcctgacctgtagcgtcagcggaggctctatctctagcggcggctatagctggtcctggattagacagcccccaggtaaaggcctcgagtatatcggctatatctactataggggcactacctactataaccctagcctgaagtctaggatcactatgagcgtggacacctctaacaatcagattagcctgaagctgactagcgtgaccgccgctgacaccgccgtctactactgcgctagagccctgactcacctcgttggagtgggctggtttgacccttggggtcaaggcactatggtcaccgtgtctagc

SEQ ID NO: 195 - protein, 453 aa, synthetic construct
  REGION 1..453: note = source = /note="Description of Artificial Sequence: Synthetic polypeptide"
QVQLQESGPGLAKPSQTLSLTCSVSGGSISSGGYSWSWIRQPPGKGLEYIGYIYYRGTTYYNPSLKSRITMSVDTSNNQISLKLTSVTAADTAVYYCARALTHLVGVGWFDPWGQGTMVTVSSASTKGPSVFPLAPSSKSTSGGTAALGCLVKDYFPEPVTVSWNSGALTSGVHTFPAVLQSSGLYSLSSVVTVPSSSLGTQTYICNVNHKPSNTKVDKRVEPKSCDKTHTCPPCPAPELLGGPSVFLFPPKPKDTLMISRTPEVTCVVVDVSHEDPEVKFNWYVDGVEVHNAKTKPREEQYNSTYRVVSVLTVLHQDWLNGKEYKCKVSNKALPAPIEKTISKAKGQPREPQVYTLPPSREEMTKNQVSLTCLVKGFYPSDIAVEWESNGQPENNYKTTPPVLDSDGSFFLYSKLTVDKSRWQQGNVFSCSVMHEALHNHYTQKSLSLSPGK

SEQ ID NO: 196 - DNA, 1359 bp, synthetic construct
  misc_feature 1..1359: note = source = /note="Description of Artificial Sequence: Synthetic polynucleotide"
  source 1..1359: mol_type = other DNA
caggtgcagctgcaagaatcaggccctggcctggctaagcctagtcagaccctgagcctgacctgtagcgtcagcggaggctctatctctagcggcggctatagctggtcctggattagacagcccccaggtaaaggcctcgagtatatcggctatatctactataggggcactacctactataaccctagcctgaagtctaggatcactatgagcgtggacacctctaacaatcagattagcctgaagctgactagcgtgaccgccgctgacaccgccgtctactactgcgctagagccctgactcacctcgttggagtgggctggtttgacccttggggtcaaggcactatggtcaccgtgtctagcgctagcactaagggcccaagtgtgtttcccctggcccccagcagcaagtctacttccggcggaactgctgccctgggttgcctggtgaaggactacttccccgagcccgtgacagtgtcctggaactctggggctctgacttccggcgtgcacaccttccccgccgtgctgcagagcagcggcctgtacagcctgagcagcgtggtgacagtgccctccagctctctgggaacccagacctatatctgcaacgtgaaccacaagcccagcaacaccaaggtggacaagagagtggagcccaagagctgcgacaagacccacacctgccccccctgcccagctccagaactgctgggagggccttccgtgttcctgttcccccccaagcccaaggacaccctgatgatcagcaggacccccgaggtgacctgcgtggtggtggacgtgtcccacgaggacccagaggtgaagttcaactggtacgtggacggcgtggaggtgcacaacgccaagaccaagcccagagaggagcagtacaacagcacctacagggtggtgtccgtgctgaccgtgctgcaccaggactggctgaacggcaaagaatacaagtgcaaagtctccaacaaggccctgccagccccaatcgaaaagacaatcagcaaggccaagggccagccacgggagccccaggtgtacaccctgccccccagccgggaggagatgaccaagaaccaggtgtccctgacctgtctggtgaagggcttctaccccagcgatatcgccgtggagtgggagagcaacggccagcccgagaacaactacaagaccacccccccagtgctggacagcgacggcagcttcttcctgtacagcaagctgaccgtggacaagtccaggtggcagcagggcaacgtgttcagctgcagcgtgatgcacgaggccctgcacaaccactacacccagaagtccctgagcctgagccccggcaag

SEQ ID NO: 197 - protein, 13 aa, synthetic construct
  REGION 1..13: note = source = /note="Description of Artificial Sequence: Synthetic peptide"
SGGSSNLGSNYVS

SEQ ID NO: 198 - protein, 7 aa, synthetic construct
  REGION 1..7: note = source = /note="Description of Artificial Sequence: Synthetic peptide"
DNNKRPS

SEQ ID NO: 199 - protein, 11 aa, synthetic construct
  REGION 1..11: note = source = /note="Description of Artificial Sequence: Synthetic peptide"
GTWDGSLSAWV

SEQ ID NO: 200 - protein, 9 aa, synthetic construct
  REGION 1..9: note = source = /note="Description of Artificial Sequence: Synthetic peptide"
GSSNLGSNY

SEQ ID NO: 201 - skipped

SEQ ID NO: 202 - protein, 8 aa, synthetic construct
  REGION 1..8: note = source = /note="Description of Artificial Sequence: Synthetic peptide"
WDGSLSAW

SEQ ID NO: 203 - protein, 110 aa, synthetic construct
  REGION 1..110: note = source = /note="Description of Artificial Sequence: Synthetic polypeptide"
QSVLTQPPSVSAAPGQKVTISCSGGSSNLGSNYVSWYQQLPGTAPKLLIYDNNKRPSGIPDRFSGSKSGTSATLGITGLQTGDEADYYCGTWDGSLSAWVFGGGTKVTVL

SEQ ID NO: 204 - DNA, 330 bp, synthetic construct
  misc_feature 1..330: note = source = /note="Description of Artificial Sequence: Synthetic polynucleotide"
  source 1..330: mol_type = other DNA
cagtcagtcctgactcagccccctagcgtcagcgccgctcccggtcaaaaagtgactattagctgtagcggcggctcctctaacctgggctctaactacgtcagctggtatcagcagctgcccggcaccgcccctaagctgctgatctacgataacaacaagcggcctagcggaatccccgataggtttagcggctctaagtcaggcactagcgctaccctgggaatcaccggcctgcagaccggcgacgaggccgactactactgtggcacctgggacggtagcctgagcgcctgggtgttcggcggaggcactaaagtcacagtgctg

SEQ ID NO: 205 - protein, 216 aa, synthetic construct
  REGION 1..216: note = source = /note="Description of Artificial Sequence: Synthetic polypeptide"
QSVLTQPPSVSAAPGQKVTISCSGGSSNLGSNYVSWYQQLPGTAPKLLIYDNNKRPSGIPDRFSGSKSGTSATLGITGLQTGDEADYYCGTWDGSLSAWVFGGGTKVTVLGQPKAAPSVTLFPPSSEELQANKATLVCLISDFYPGAVTVAWKADSSPVKAGVETTTPSKQSNNKYAASSYLSLTPEQWKSHRSYSCQVTHEGSTVEKTVAPTECS

SEQ ID NO: 206 - DNA, 648 bp, synthetic construct
  misc_feature 1..648: note = source = /note="Description of Artificial Sequence: Synthetic polynucleotide"
  source 1..648: mol_type = other DNA
cagtcagtcctgactcagccccctagcgtcagcgccgctcccggtcaaaaagtgactattagctgtagcggcggctcctctaacctgggctctaactacgtcagctggtatcagcagctgcccggcaccgcccctaagctgctgatctacgataacaacaagcggcctagcggaatccccgataggtttagcggctctaagtcaggcactagcgctaccctgggaatcaccggcctgcagaccggcgacgaggccgactactactgtggcacctgggacggtagcctgagcgcctgggtgttcggcggaggcactaaagtcacagtgctgggtcaacctaaggctgcccccagcgtgaccctgttcccccccagcagcgaggagctgcaggccaacaaggccaccctggtgtgcctgatcagcgacttctacccaggcgccgtgaccgtggcctggaaggccgacagcagccccgtgaaggccggcgtggagaccaccacccccagcaagcagagcaacaacaagtacgccgccagcagctacctgagcctgacccccgagcagtggaagagccacaggtcctacagctgccaggtgacccacgagggcagcaccgtggaaaagaccgtggccccaaccgagtgcagc

SEQ ID NO: 207 - protein, 7 aa, synthetic construct
  REGION 1..7: note = source = /note="Description of Artificial Sequence: Synthetic peptide"
SGGYSWS

SEQ ID NO: 208 - protein, 16 aa, synthetic construct
  REGION 1..16: note = source = /note="Description of Artificial Sequence: Synthetic peptide"
YIYYRGTTYYNPSLKS

SEQ ID NO: 209 - protein, 13 aa, synthetic construct
  REGION 1..13: note = source = /note="Description of Artificial Sequence: Synthetic peptide"
ALTHLVGVGWFDP

SEQ ID NO: 210 - protein, 9 aa, synthetic construct
  REGION 1..9: note = source = /note="Description of Artificial Sequence: Synthetic peptide"
GGSISSGGY

SEQ ID NO: 211 - protein, 5 aa, synthetic construct
  REGION 1..5: note = source = /note="Description of Artificial Sequence: Synthetic peptide"
YYRGT

SEQ ID NO: 212 - protein, 13 aa, synthetic construct
  REGION 1..13: note = source = /note="Description of Artificial Sequence: Synthetic peptide"
ALTHLVGVGWFDP

SEQ ID NO: 213 - protein, 123 aa, synthetic construct
  REGION 1..123: note = source = /note="Description of Artificial Sequence: Synthetic polypeptide"
QVQLQESGPGLVKPSQTLSLTCTVSGGSISSGGYSWSWIRQPPGKGLEYIGYIYYRGTTYYNPSLKSRVTISVDTSNNQISLKLSSVTAADTAVYYCARALTHLVGVGWFDPWGQGTMVTVSS

SEQ ID NO: 214 - DNA, 369 bp, synthetic construct
  misc_feature 1..369: note = source = /note="Description of Artificial Sequence: Synthetic polynucleotide"
  source 1..369: mol_type = other DNA
caggtgcagctgcaagaatcaggccctggcctggtcaagcctagtcagaccctgagcctgacctgcaccgtcagcggaggctctatctctagcggcggctatagctggtcctggattagacagcccccaggtaaaggcctcgagtatatcggctatatctactataggggcactacctactataaccctagcctgaagtctagggtcacaattagcgtggacacctctaacaatcagattagcctgaagctgtctagcgtgaccgccgctgacaccgccgtctactactgcgctagagccctgactcacctcgtcggagtgggctggtttgacccttggggtcaaggcactatggtcaccgtgtctagc

SEQ ID NO: 215 - protein, 453 aa, synthetic construct
  REGION 1..453: note = source = /note="Description of Artificial Sequence: Synthetic polypeptide"
QVQLQESGPGLVKPSQTLSLTCTVSGGSISSGGYSWSWIRQPPGKGLEYIGYIYYRGTTYYNPSLKSRVTISVDTSNNQISLKLSSVTAADTAVYYCARALTHLVGVGWFDPWGQGTMVTVSSASTKGPSVFPLAPSSKSTSGGTAALGCLVKDYFPEPVTVSWNSGALTSGVHTFPAVLQSSGLYSLSSVVTVPSSSLGTQTYICNVNHKPSNTKVDKRVEPKSCDKTHTCPPCPAPELLGGPSVFLFPPKPKDTLMISRTPEVTCVVVDVSHEDPEVKFNWYVDGVEVHNAKTKPREEQYNSTYRVVSVLTVLHQDWLNGKEYKCKVSNKALPAPIEKTISKAKGQPREPQVYTLPPSREEMTKNQVSLTCLVKGFYPSDIAVEWESNGQPENNYKTTPPVLDSDGSFFLYSKLTVDKSRWQQGNVFSCSVMHEALHNHYTQKSLSLSPGK

SEQ ID NO: 216 - DNA, 1359 bp, synthetic construct
  misc_feature 1..1359: note = source = /note="Description of Artificial Sequence: Synthetic polynucleotide"
  source 1..1359: mol_type = other DNA
caggtgcagctgcaagaatcaggccctggcctggtcaagcctagtcagaccctgagcctgacctgcaccgtcagcggaggctctatctctagcggcggctatagctggtcctggattagacagcccccaggtaaaggcctcgagtatatcggctatatctactataggggcactacctactataaccctagcctgaagtctagggtcacaattagcgtggacacctctaacaatcagattagcctgaagctgtctagcgtgaccgccgctgacaccgccgtctactactgcgctagagccctgactcacctcgtcggagtgggctggtttgacccttggggtcaaggcactatggtcaccgtgtctagcgctagcactaagggcccaagtgtgtttcccctggcccccagcagcaagtctacttccggcggaactgctgccctgggttgcctggtgaaggactacttccccgagcccgtgacagtgtcctggaactctggggctctgacttccggcgtgcacaccttccccgccgtgctgcagagcagcggcctgtacagcctgagcagcgtggtgacagtgccctccagctctctgggaacccagacctatatctgcaacgtgaaccacaagcccagcaacaccaaggtggacaagagagtggagcccaagagctgcgacaagacccacacctgccccccctgcccagctccagaactgctgggagggccttccgtgttcctgttcccccccaagcccaaggacaccctgatgatcagcaggacccccgaggtgacctgcgtggtggtggacgtgtcccacgaggacccagaggtgaagttcaactggtacgtggacggcgtggaggtgcacaacgccaagaccaagcccagagaggagcagtacaacagcacctacagggtggtgtccgtgctgaccgtgctgcaccaggactggctgaacggcaaagaatacaagtgcaaagtctccaacaaggccctgccagccccaatcgaaaagacaatcagcaaggccaagggccagccacgggagccccaggtgtacaccctgccccccagccgggaggagatgaccaagaaccaggtgtccctgacctgtctggtgaagggcttctaccccagcgatatcgccgtggagtgggagagcaacggccagcccgagaacaactacaagaccacccccccagtgctggacagcgacggcagcttcttcctgtacagcaagctgaccgtggacaagtccaggtggcagcagggcaacgtgttcagctgcagcgtgatgcacgaggccctgcacaaccactacacccagaagtccctgagcctgagccccggcaag

SEQ ID NO: 217 - protein, 13 aa, synthetic construct
  REGION 1..13: note = source = /note="Description of Artificial Sequence: Synthetic peptide"
SGGSSNLGSNYVS

SEQ ID NO: 218 - protein, 7 aa, synthetic construct
  REGION 1..7: note = source = /note="Description of Artificial Sequence: Synthetic peptide"
DNNKRPS

SEQ ID NO: 219 - protein, 11 aa, synthetic construct
  REGION 1..11: note = source = /note="Description of Artificial Sequence: Synthetic peptide"
GTWDGSLSAWV

SEQ ID NO: 220 - protein, 9 aa, synthetic construct
  REGION 1..9: note = source = /note="Description of Artificial Sequence: Synthetic peptide"
GSSNLGSNY

SEQ ID NO: 221 - skipped

SEQ ID NO: 222 - protein, 8 aa, synthetic construct
  REGION 1..8: note = source = /note="Description of Artificial Sequence: Synthetic peptide"
WDGSLSAW

SEQ ID NO: 223 - protein, 110 aa, synthetic construct; identical to SEQ ID NO: 203
  REGION 1..110: note = source = /note="Description of Artificial Sequence: Synthetic polypeptide"

SEQ ID NO: 224 - DNA, 330 bp, synthetic construct; identical to SEQ ID NO: 204
  misc_feature 1..330: note = source = /note="Description of Artificial Sequence: Synthetic polynucleotide"
  source 1..330: mol_type = other DNA

SEQ ID NO: 225 - protein, 216 aa, synthetic construct; identical to SEQ ID NO: 205
  REGION 1..216: note = source = /note="Description of Artificial Sequence: Synthetic polypeptide"

SEQ ID NO: 226 - DNA, 648 bp, synthetic construct; identical to SEQ ID NO: 206
  misc_feature 1..648: note = source = /note="Description of Artificial Sequence: Synthetic polynucleotide"
  source 1..648: mol_type = other DNA

SEQ ID NO: 227 - protein, 5 aa, synthetic construct
  REGION 1..5: note = source = /note="Description of Artificial Sequence: Synthetic peptide"
AYYWT

SEQ ID NO: 228 - protein, 16 aa, synthetic construct
  REGION 1..16: note = source = /note="Description of Artificial Sequence: Synthetic peptide"
YISHSGSTNYNPSLKS

SEQ ID NO: 229 - protein, 16 aa, synthetic construct
  REGION 1..16: note = source = /note="Description of Artificial Sequence: Synthetic peptide"
LGDTASLSRFYYYIDV

SEQ ID NO: 230 - protein, 7 aa, synthetic construct
  REGION 1..7: note = source = /note="Description of Artificial Sequence: Synthetic peptide"
GGSTSAY

SEQ ID NO: 231 - protein, 5 aa, synthetic construct
  REGION 1..5: note = source = /note="Description of Artificial Sequence: Synthetic peptide"
SHSGS

SEQ ID NO: 232 - protein, 16 aa, synthetic construct
  REGION 1..16: note = source = /note="Description of Artificial Sequence: Synthetic peptide"
LGDTASLSRFYYYIDV

SEQ ID NO: 233 - protein, 124 aa, synthetic construct
  REGION 1..124: note = source = /note="Description of Artificial Sequence: Synthetic polypeptide"
QVQLVQSGPGLVKPSETLSLTCTVSGGSTSAYYWTWIRQPPGKGLEWIGYISHSGSTNYNPSLKSRVTISADTSKNQLSLKVNSVTAADTAVYYCARLGDTASLSRFYYYIDVWGKGTTVTVSS

SEQ ID NO: 234 - DNA, 372 bp, synthetic construct
  misc_feature 1..372: note = source = /note="Description of Artificial Sequence: Synthetic polynucleotide"
  source 1..372: mol_type = other DNA
caggtgcagctggtgcagtctggcccaggactggtgaagccttcggagaccctgtccctcacctgcactgtctctggtggctccaccagtgcttactactggacctggattcggcagcccccagggaagggactggagtggattgggtatatctctcacagtgggagcaccaactacaacccctccctcaagagtcgagtcaccatatcagcagacacgtccaagaaccagctctccctgaaggtgaactctgtgaccgccgcagacacggccgtgtattactgtgcgagacttggggatacagcttcacttagccgcttctactactacattgacgtctggggcaaagggaccacggtcaccgtctcctca

SEQ ID NO: 235 - protein, 454 aa, synthetic construct
  REGION 1..454: note = source = /note="Description of Artificial Sequence: Synthetic polypeptide"
QVQLVQSGPGLVKPSETLSLTCTVSGGSTSAYYWTWIRQPPGKGLEWIGYISHSGSTNYNPSLKSRVTISADTSKNQLSLKVNSVTAADTAVYYCARLGDTASLSRFYYYIDVWGKGTTVTVSSASTKGPSVFPLAPSSKSTSGGTAALGCLVKDYFPEPVTVSWNSGALTSGVHTFPAVLQSSGLYSLSSVVTVPSSSLGTQTYICNVNHKPSNTKVDKRVEPKSCDKTHTCPPCPAPELLGGPSVFLFPPKPKDTLMISRTPEVTCVVVDVSHEDPEVKFNWYVDGVEVHNAKTKPREEQYNSTYRVVSVLTVLHQDWLNGKEYKCKVSNKALPAPIEKTISKAKGQPREPQVYTLPPSREEMTKNQVSLTCLVKGFYPSDIAVEWESNGQPENNYKTTPPVLDSDGSFFLYSKLTVDKSRWQQGNVFSCSVMHEALHNHYTQKSLSLSPGK

SEQ ID NO: 236 - DNA, 1362 bp, synthetic construct
  misc_feature 1..1362: note = source = /note="Description of Artificial Sequence: Synthetic polynucleotide"
  source 1..1362: mol_type = other DNA
caggtgcagctggtgcagtctggcccaggactggtgaagccttcggagaccctgtccctcacctgcactgtctctggtggctccaccagtgcttactactggacctggattcggcagcccccagggaagggactggagtggattgggtatatctctcacagtgggagcaccaactacaacccctccctcaagagtcgagtcaccatatcagcagacacgtccaagaaccagctctccctgaaggtgaactctgtgaccgccgcagacacggccgtgtattactgtgcgagacttggggatacagcttcacttagccgcttctactactacattgacgtctggggcaaagggaccacggtcaccgtctcctcagctagcaccaagggcccatcggtcttccccctggcaccctcctccaagagcacctctgggggcacagcggccctgggctgcctggtcaaggactacttccccgaaccggtgacggtgtcgtggaactcaggcgccctgaccagcggcgtgcacaccttcccggctgtcctacagtcctcaggactctactccctcagcagcgtggtgaccgtgccctccagcagcttgggcacccagacctacatctgcaacgtgaatcacaagcccagcaacaccaaggtggacaagagagttgagcccaaatcttgtgacaaaactcacacatgcccaccgtgcccagcacctgaactcctggggggaccgtcagtcttcctcttccccccaaaacccaaggacaccctcatgatctcccggacccctgaggtcacatgcgtggtggtggacgtgagccacgaagaccctgaggtcaagttcaactggtacgtggacggcgtggaggtgcataatgccaagacaaagccgcgggaggagcagtacaacagcacgtaccgtgtggtcagcgtcctcaccgtcctgcaccaggactggctgaatggcaaggagtacaagtgcaaggtctccaacaaagccctcccagcccccatcgagaaaaccatctccaaagccaaagggcagccccgagaaccacaggtgtacaccctgcccccatcccgggaggagatgaccaagaaccaggtcagcctgacctgcctggtcaaaggcttctatcccagcgacatcgccgtggagtgggagagcaatgggcagccggagaacaactacaagaccacgcctcccgtgctggactccgacggctccttcttcctctacagcaagctcaccgtggacaagagcaggtggcagcaggggaacgtcttctcatgctccgtgatgcatgaggctctgcacaaccactacacgcagaagagcctctccctgtctccgggtaaa

SEQ ID NO: 237 - protein, 12 aa, synthetic construct
  REGION 1..12: note = source = /note="Description of Artificial Sequence: Synthetic peptide"
RASQSVSSNYLA

SEQ ID NO: 238 - protein, 7 aa, synthetic construct
  REGION 1..7: note = source = /note="Description of Artificial Sequence: Synthetic peptide"
GASSRAT

SEQ ID NO: 239 - protein, 10 aa, synthetic construct
  REGION 1..10: note = source = /note="Description of Artificial Sequence: Synthetic peptide"
QQYGSSPPYT

SEQ ID NO: 240 - protein, 8 aa, synthetic construct
  REGION 1..8: note = source = /note="Description of Artificial Sequence: Synthetic peptide"
SQSVSSNY

SEQ ID NO: 241 - skipped

SEQ ID NO: 242 - protein, 7 aa, synthetic construct
  REGION 1..7: note = source = /note="Description of Artificial Sequence: Synthetic peptide"
YGSSPPY

SEQ ID NO: 243 - protein, 109 aa, synthetic construct
  REGION 1..109: note = source = /note="Description of Artificial Sequence: Synthetic polypeptide"
EIVMTQSPDTLSLSPGERATLSCRASQSVSSNYLAWYQQKPGEAPRLLIYGASSRATGIPDRFSGSGSGTDFTLTISRLEPEDFAVYYCQQYGSSPPYTFGQGTRLEIK

SEQ ID NO: 244 - DNA, 328 bp, synthetic construct
  misc_feature 1..328: note = source = /note="Description of Artificial Sequence: Synthetic polynucleotide"
  source 1..328: mol_type = other DNA
gaaattgtaatgacgcagtctccagacaccctgtctttgtctccaggggaaagagccaccctctcctgcagggccagtcagagtgttagcagcaactacttagcctggtaccagcagaaacctggcgaggctcccaggctcctcatctatggtgcatccagcagggccactggcatcccagacaggttcagtggcagtgggtctgggacagacttcactctcaccatcagcagactggagcctgaagattttgcagtgtattactgtcagcagtatggtagctcacctccgtacacttttggccaggggacacgactggagattaaac

SEQ ID NO: 245 - protein, 216 aa, synthetic construct
  REGION 1..216: note = source = /note="Description of Artificial Sequence: Synthetic polypeptide"
EIVMTQSPDTLSLSPGERATLSCRASQSVSSNYLAWYQQKPGEAPRLLIYGASSRATGIPDRFSGSGSGTDFTLTISRLEPEDFAVYYCQQYGSSPPYTFGQGTRLEIKRTVAAPSVFIFPPSDEQLKSGTASVVCLLNNFYPREAKVQWKVDNALQSGNSQESVTEQDSKDSTYSLSSTLTLSKADYEKHKVYACEVTHQGLSSPVTKSFNRGEC

SEQ ID NO: 246 - DNA, 648 bp, synthetic construct
  misc_feature 1..648: note = source = /note="Description of Artificial Sequence: Synthetic polynucleotide"
  source 1..648: mol_type = other DNA
gaaattgtaatgacgcagtctccagacaccctgtctttgtctccaggggaaagagccaccctctcctgcagggccagtcagagtgttagcagcaactacttagcctggtaccagcagaaacctggcgaggctcccaggctcctcatctatggtgcatccagcagggccactggcatcccagacaggttcagtggcagtgggtctgggacagacttcactctcaccatcagcagactggagcctgaagattttgcagtgtattactgtcagcagtatggtagctcacctccgtacacttttggccaggggacacgactggagattaaacgtacggtggctgcaccatctgtcttcatcttcccgccatctgatgagcagttgaaatctggaactgcctctgttgtgtgcctgctgaataacttctatccccgcgaggccaaagtacagtggaaggtggataacgccctccaatcgggtaactcccaggagagtgtcacagagcaggacagcaaggacagcacctacagcctcagcagcaccctgacgctgagcaaagcagactacgagaaacacaaagtctacgcctgcgaagtcacccatcagggcctgagctcgcccgtcacaaagagcttcaaccgcggagagtgt

SEQ ID NO: 247 - protein, 5 aa, synthetic construct
  REGION 1..5: note = source = /note="Description of Artificial Sequence: Synthetic peptide"
RNYMS

SEQ ID NO: 248 - protein, 16 aa, synthetic construct
  REGION 1..16: note = source = /note="Description of Artificial Sequence: Synthetic peptide"
GIYSGGSTYYADSVKG

SEQ ID NO: 249 - protein, 13 aa, synthetic construct
  REGION 1..13: note = source = /note="Description of Artificial Sequence: Synthetic peptide"
EDEFWSGYSAGVD

SEQ ID NO: 250 - protein, 7 aa, synthetic construct
  REGION 1..7: note = source = /note="Description of Artificial Sequence: Synthetic peptide"
GFTVRRN

SEQ ID NO: 251 - protein, 5 aa, synthetic construct
  REGION 1..5: note = source = /note="Description of Artificial Sequence: Synthetic peptide"
YSGGS

SEQ ID NO: 252 - protein, 13 aa, synthetic construct
  REGION 1..13: note = source = /note="Description of Artificial Sequence: Synthetic peptide"
EDEFWSGYSAGVD

SEQ ID NO: 253 - protein, 121 aa, synthetic construct
  REGION 1..121: note = source = /note="Description of Artificial Sequence: Synthetic polypeptide"
EVQLVETGGGLVQPGGSLRLSCAASGFTVRRNYMSWVRQAPGKGLEWVSGIYSGGSTYYADSVKGRFTISRDYSKNTLSLQMNTLRVEDTAVYFCAREDEFWSGYSAGVDWGQGTLVTVSS

SEQ ID NO: 254 - DNA, 364 bp, synthetic construct
  misc_feature 1..364: note = source = /note="Description of Artificial Sequence: Synthetic polynucleotide"
  source 1..364: mol_type = other DNA
gaggtgcagctggtggagactggaggaggcttggtccagccgggggggtccctgagactctcatgtgcagcctctggattcaccgtcagacgcaattacatgagttgggtccgccaggctccggggaagggactggagtgggtctcagggatctacagtggtggtagcacatactacgcagactccgtgaagggccgattcaccatctccagagactattccaagaacacactgtctcttcaaatgaacaccctgagagtcgaggacacggccgtgtatttctgtgcgagagaagacgaattttggagcgggtattccgctggggtcgactggggccagggaaccctggtcaccgtctcctcag

SEQ ID NO: 255 - protein, 451 aa, synthetic construct
  REGION 1..451: note = source = /note="Description of Artificial Sequence: Synthetic polypeptide"
EVQLVETGGGLVQPGGSLRLSCAASGFTVRRNYMSWVRQAPGKGLEWVSGIYSGGSTYYADSVKGRFTISRDYSKNTLSLQMNTLRVEDTAVYFCAREDEFWSGYSAGVDWGQGTLVTVSSASTKGPSVFPLAPSSKSTSGGTAALGCLVKDYFPEPVTVSWNSGALTSGVHTFPAVLQSSGLYSLSSVVTVPSSSLGTQTYICNVNHKPSNTKVDKRVEPKSCDKTHTCPPCPAPELLGGPSVFLFPPKPKDTLMISRTPEVTCVVVDVSHEDPEVKFNWYVDGVEVHNAKTKPREEQYNSTYRVVSVLTVLHQDWLNGKEYKCKVSNKALPAPIEKTISKAKGQPREPQVYTLPPSREEMTKNQVSLTCLVKGFYPSDIAVEWESNGQPENNYKTTPPVLDSDGSFFLYSKLTVDKSRWQQGNVFSCSVMHEALHNHYTQKSLSLSPGK

SEQ ID NO: 256 - DNA, 1353 bp, synthetic construct
  misc_feature 1..1353: note = source = /note="Description of Artificial Sequence: Synthetic polynucleotide"
  source 1..1353: mol_type = other DNA
gaggtgcagctggtggagactggaggaggcttggtccagccgggggggtccctgagactctcatgtgcagcctctggattcaccgtcagacgcaattacatgagttgggtccgccaggctccggggaagggactggagtgggtctcagggatctacagtggtggtagcacatactacgcagactccgtgaagggccgattcaccatctccagagactattccaagaacacactgtctcttcaaatgaacaccctgagagtcgaggacacggccgtgtatttctgtgcgagagaagacgaattttggagcgggtattccgctggggtcgactggggccagggaaccctggtcaccgtctcctcagctagcaccaagggcccatcggtcttccccctggcaccctcctccaagagcacctctgggggcacagcggccctgggctgcctggtcaaggactacttccccgaaccggtgacggtgtcgtggaactcaggcgccctgaccagcggcgtgcacaccttcccggctgtcctacagtcctcaggactctactccctcagcagcgtggtgaccgtgccctccagcagcttgggcacccagacctacatctgcaacgtgaatcacaagcccagcaacaccaaggtggacaagagagttgagcccaaatcttgtgacaaaactcacacatgcccaccgtgcccagcacctgaactcctggggggaccgtcagtcttcctcttccccccaaaacccaaggacaccctcatgatctcccggacccctgaggtcacatgcgtggtggtggacgtgagccacgaagaccctgaggtcaagttcaactggtacgtggacggcgtggaggtgcataatgccaagacaaagccgcgggaggagcagtacaacagcacgtaccgtgtggtcagcgtcctcaccgtcctgcaccaggactggctgaatggcaaggagtacaagtgcaaggtctccaacaaagccctcccagcccccatcgagaaaaccatctccaaagccaaagggcagccccgagaaccacaggtgtacaccctgcccccatcccgggaggagatgaccaagaaccaggtcagcctgacctgcctggtcaaaggcttctatcccagcgacatcgccgtggagtgggagagcaatgggcagccggagaacaactacaagaccacgcctcccgtgctggactccgacggctccttcttcctctacagcaagctcaccgtggacaagagcaggtggcagcaggggaacgtcttctcatgctccgtgatgcatgaggctctgcacaaccactacacgcagaagagcctctccctgtctccgggtaaa

SEQ ID NO: 257 - protein, 11 aa, synthetic construct
  REGION 1..11: note = source = /note="Description of Artificial Sequence: Synthetic peptide"
RASQSISSYLN

SEQ ID NO: 258 - protein, 7 aa, synthetic construct
  REGION 1..7: note = source = /note="Description of Artificial Sequence: Synthetic peptide"
AASSLQS

SEQ ID NO: 259 - protein, 9 aa, synthetic construct
  REGION 1..9: note = source = /note="Description of Artificial Sequence: Synthetic peptide"
QQSYNTPRT

SEQ ID NO: 260 - protein, 7 aa, synthetic construct
  REGION 1..7: note = source = /note="Description of Artificial Sequence: Synthetic peptide"
SQSISSY

SEQ ID NO: 261 - skipped

SEQ ID NO: 262 - protein, 6 aa, synthetic construct
  REGION 1..6: note = source = /note="Description of Artificial Sequence: Synthetic peptide"
SYNTPR

SEQ ID NO: 263 - protein, 107 aa, synthetic construct
  REGION 1..107: note = source = /note="Description of Artificial Sequence: Synthetic polypeptide"
DIRLTQSPSSLSASVGDRVTITCRASQSISSYLNWYQQKPGKAPKLLIYAASSLQSGVPSRFSGSGSGTDFTLTISSLQPEDFATYYCQQSYNTPRTFGQGTKVEIK

SEQ ID NO: 264 - DNA, 323 bp, synthetic construct
  misc_feature 1..323: note = source = /note="Description of Artificial Sequence: Synthetic polynucleotide"
  source 1..323: mol_type = other DNA
gacatccggttgacccagtctccatcctccctgtctgcatctgtaggagacagagtcaccatcacttgccgggcaagtcagagcattagcagctatttgaattggtatcagcagaaaccagggaaagcccctaagctcctgatctatgctgcatccagtttgcaaagtggggtcccatcaaggttcagtggcagtggatctgggacagatttcactctcaccatcagcagtctgcaacctgaagattttgcaacttactactgtcaacagagttacaatacccctcgaacgttcggccaagggaccaaggtggagatcaaacg

SEQ ID NO: 265 - protein, 214 aa, synthetic construct
  REGION 1..214: note = source = /note="Description of Artificial Sequence: Synthetic polypeptide"
DIRLTQSPSSLSASVGDRVTITCRASQSISSYLNWYQQKPGKAPKLLIYAASSLQSGVPSRFSGSGSGTDFTLTISSLQPEDFATYYCQQSYNTPRTFGQGTKVEIKRTVAAPSVFIFPPSDEQLKSGTASVVCLLNNFYPREAKVQWKVDNALQSGNSQESVTEQDSKDSTYSLSSTLTLSKADYEKHKVYACEVTHQGLSSPVTKSFNRGEC

SEQ ID NO: 266 - DNA, 642 bp, synthetic construct
  misc_feature 1..642: note = source = /note="Description of Artificial Sequence: Synthetic polynucleotide"
  source 1..642: mol_type = other DNA
gacatccggttgacccagtctccatcctccctgtctgcatctgtaggagacagagtcaccatcacttgccgggcaagtcagagcattagcagctatttgaattggtatcagcagaaaccagggaaagcccctaagctcctgatctatgctgcatccagtttgcaaagtggggtcccatcaaggttcagtggcagtggatctgggacagatttcactctcaccatcagcagtctgcaacctgaagattttgcaacttactactgtcaacagagttacaatacccctcgaacgttcggccaagggaccaaggtggagatcaaacgtacggtggctgcaccatctgtcttcatcttcccgccatctgatgagcagttgaaatctggaactgcctctgttgtgtgcctgctgaataacttctatccccgcgaggccaaagtacagtggaaggtggataacgccctccaatcgggtaactcccaggagagtgtcacagagcaggacagcaaggacagcacctacagcctcagcagcaccctgacgctgagcaaagcagactacgagaaacacaaagtctacgcctgcgaagtcacccatcagggcctgagctcgcccgtcacaaagagcttcaaccgcggagagtgt

SEQ ID NO: 267 - protein, 5 aa, synthetic construct
  REGION 1..5: note = source = /note="Description of Artificial Sequence: Synthetic peptide"
RNYMS

SEQ ID NO: 268 - protein, 16 aa, synthetic construct
  REGION 1..16: note = source = /note="Description of Artificial Sequence: Synthetic peptide"
GIYSGGSTYYADSVKG

SEQ ID NO: 269 - protein, 13 aa, synthetic construct
  REGION 1..13: note = source = /note="Description of Artificial Sequence: Synthetic peptide"
EDEFWSGYSAGVD

SEQ ID NO: 270 - protein, 7 aa, synthetic construct
  REGION 1..7: note = source = /note="Description of Artificial Sequence: Synthetic peptide"
GFTVSRN

SEQ ID NO: 271 - protein, 5 aa, synthetic construct
  REGION 1..5: note = source = /note="Description of Artificial Sequence: Synthetic peptide"
YSGGS

SEQ ID NO: 272 - protein, 13 aa, synthetic construct
  REGION 1..13: note = source = /note="Description of Artificial Sequence: Synthetic peptide"
EDEFWSGYSAGVD

SEQ ID NO: 273 - protein, 121 aa, synthetic construct
  REGION 1..121: note = source = /note="Description of Artificial Sequence: Synthetic polypeptide"
QVQLVESGGGLVQPGGSLRLSCAASGFTVSRNYMSWVRQAPGKGLEWVSGIYSGGSTYYADSVKGRFTISRDYSKNTLSLQMNTLRVEDTAVYFCAREDEFWSGYSAGVDWGQGTLVTVSS

SEQ ID NO: 274 - DNA, 365 bp, synthetic construct
  misc_feature 1..365: note = source = /note="Description of Artificial Sequence: Synthetic polynucleotide"
  source 1..365: mol_type = other DNA
caggtgcagctggtggaatctggaggaggcttggtccagcctggggggtccctgagactctcatgtgcagcctctggattcaccgtcagtcgcaattacatgagttgggtccgccaggctccggggaagggactggagtgggtctcagggatttacagtggtggtagcacatactacgcagactccgtgaagggccgattcaccatctccagagactattccaagaacacactgtctcttcaaatgaacaccctgagagtcgaggacacggccgtgtatttctgtgcgagagaagacgaattttggagtgggtattccgctggggtcgactggggccagggaaccctggtcaccgtctcctcagc

SEQ ID NO: 275 - protein, 451 aa, synthetic construct
  REGION 1..451: note = source = /note="Description of Artificial Sequence: Synthetic polypeptide"
QVQLVESGGGLVQPGGSLRLSCAASGFTVSRNYMSWVRQAPGKGLEWVSGIYSGGSTYYADSVKGRFTISRDYSKNTLSLQMNTLRVEDTAVYFCAREDEFWSGYSAGVDWGQGTLVTVSSASTKGPSVFPLAPSSKSTSGGTAALGCLVKDYFPEPVTVSWNSGALTSGVHTFPAVLQSSGLYSLSSVVTVPSSSLGTQTYICNVNHKPSNTKVDKRVEPKSCDKTHTCPPCPAPELLGGPSVFLFPPKPKDTLMISRTPEVTCVVVDVSHEDPEVKFNWYVDGVEVHNAKTKPREEQYNSTYRVVSVLTVLHQDWLNGKEYKCKVSNKALPAPIEKTISKAKGQPREPQVYTLPPSREEMTKNQVSLTCLVKGFYPSDIAVEWESNGQPENNYKTTPPVLDSDGSFFLYSKLTVDKSRWQQGNVFSCSVMHEALHNHYTQKSLSLSPGK

SEQ ID NO: 276 - DNA, 1353 bp, synthetic construct
  misc_feature 1..1353: note = source = /note="Description of Artificial Sequence: Synthetic polynucleotide"
  source 1..1353: mol_type = other DNA
caggtgcagctggtggaatctggaggaggcttggtccagcctggggggtccctgagactctcatgtgcagcctctggattcaccgtcagtcgcaattacatgagttgggtccgccaggctccggggaagggactggagtgggtctcagggatttacagtggtggtagcacatactacgcagactccgtgaagggccgattcaccatctccagagactattccaagaacacactgtctcttcaaatgaacaccctgagagtcgaggacacggccgtgtatttctgtgcgagagaagacgaattttggagtgggtattccgctggggtcgactggggccagggaaccctggtcaccgtctcctcagctagcaccaagggcccatcggtcttccccctggcaccctcctccaagagcacctctgggggcacagcggccctgggctgcctggtcaaggactacttccccgaaccggtgacggtgtcgtggaactcaggcgccctgaccagcggcgtgcacaccttcccggctgtcctacagtcctcaggactctactccctcagcagcgtggtgaccgtgccctccagcagcttgggcacccagacctacatctgcaacgtgaatcacaagcccagcaacaccaaggtggacaagagagttgagcccaaatcttgtgacaaaactcacacatgcccaccgtgcccagcacctgaactcctggggggaccgtcagtcttcctcttccccccaaaacccaaggacaccctcatgatctcccggacccctgaggtcacatgcgtggtggtggacgtgagccacgaagaccctgaggtcaagttcaactggtacgtggacggcgtggaggtgcataatgccaagacaaagccgcgggaggagcagtacaacagcacgtaccgtgtggtcagcgtcctcaccgtcctgcaccaggactggctgaatggcaaggagtacaagtgcaaggtctccaacaaagccctcccagcccccatcgagaaaaccatctccaaagccaaagggcagccccgagaaccacaggtgtacaccctgcccccatcccgggaggagatgaccaagaaccaggtcagcctgacctgcctggtcaaaggcttctatcccagcgacatcgccgtggagtgggagagcaatgggcagccggagaacaactacaagaccacgcctcccgtgctggactccgacggctccttcttcctctacagcaagctcaccgtggacaagagcaggtggcagcaggggaacgtcttctcatgctccgtgatgcatgaggctctgcacaaccactacacgcagaagagcctctccctgtctccgggtaaa

SEQ ID NO: 277 - protein, 11 aa, synthetic construct
  REGION 1..11: note = source = /note="Description of Artificial Sequence: Synthetic peptide"
RASQSISSYLN

SEQ ID NO: 278 - protein, 7 aa, synthetic construct
  REGION 1..7: note = source = /note="Description of Artificial Sequence: Synthetic peptide"
AASSLQS

SEQ ID NO: 279 - protein, 9 aa, synthetic construct
  REGION 1..9: note = source = /note="Description of Artificial Sequence: Synthetic peptide"
QQSYSTPRT

SEQ ID NO: 280 - protein, 7 aa, synthetic construct
  REGION 1..7: note = source = /note="Description of Artificial Sequence: Synthetic peptide"
SQSISSY

SEQ ID NO: 281 - skipped

SEQ ID NO: 282 - protein, 6 aa, synthetic construct
  REGION 1..6: note = source = /note="Description of Artificial Sequence: Synthetic peptide"
SYSTPR

SEQ ID NO: 283 - protein, 107 aa, synthetic construct
  REGION 1..107: note = source = /note="Description of Artificial Sequence: Synthetic polypeptide"
DIRMTQSPSSLSASVGDRVTITCRASQSISSYLNWYQQKPGKAPTLLIYAASSLQSGVPSRFSGSGSGTDFTLTISSLQPEDFATYYCQQSYSTPRTFGQGTKVEIK

SEQ ID NO: 284 - DNA, 322 bp, synthetic construct
  misc_feature 1..322: note = source = /note="Description of Artificial Sequence: Synthetic polynucleotide"
  source 1..322: mol_type = other DNA
gacatccggatgacccagtctccatcctccctgtctgcatctgtaggagacagagtcaccatcacttgccgggcaagtcagagcattagcagctatttaaattggtatcagcagaaaccagggaaagcccctacgctcctgatctatgctgcatccagtttgcaaagtggggtcccatcaaggttcagtggcagtggatctgggacagatttcactctcaccatcagcagtctgcaacctgaagattttgcaacttactactgtcaacagagttacagtacccctcggacgttcggccaagggaccaaggtggagatcaaac

SEQ ID NO: 285 - protein, 214 aa, synthetic construct
  REGION 1..214: note = source = /note="Description of Artificial Sequence: Synthetic polypeptide"
DIRMTQSPSSLSASVGDRVTITCRASQSISSYLNWYQQKPGKAPTLLIYAASSLQSGVPSRFSGSGSGTDFTLTISSLQPEDFATYYCQQSYSTPRTFGQGTKVEIKRTVAAPSVFIFPPSDEQLKSGTASVVCLLNNFYPREAKVQWKVDNALQSGNSQESVTEQDSKDSTYSLSSTLTLSKADYEKHKVYACEVTHQGLSSPVTKSFNRGEC

SEQ ID NO: 286 - DNA, 642 bp, synthetic construct
  misc_feature 1..642: note = source = /note="Description of Artificial Sequence: Synthetic polynucleotide"
  source 1..642: mol_type = other DNA
gacatccggatgacccagtctccatcctccctgtctgcatctgtaggagacagagtcaccatcacttgccgggcaagtcagagcattagcagctatttaaattggtatcagcagaaaccagggaaagcccctacgctcctgatctatgctgcatccagtttgcaaagtggggtcccatcaaggttcagtggcagtggatctgggacagatttcactctcaccatcagcagtctgcaacctgaagattttgcaacttactactgtcaacagagttacagtacccctcggacgttcggccaagggaccaaggtggagatcaaacgtacggtggctgcaccatctgtcttcatcttcccgccatctgatgagcagttgaaatctggaactgcctctgttgtgtgcctgctgaataacttctatccccgcgaggccaaagtacagtggaaggtggataacgccctccaatcgggtaactcccaggagagtgtcacagagcaggacagcaaggacagcacctacagcctcagcagcaccctgacgctgagcaaagcagactacgagaaacacaaagtctacgcctgcgaagtcacccatcagggcctgagctcgcccgtcacaaagagcttcaaccgcggagagtgt

SEQ ID NO: 287 - protein, 5 aa, synthetic construct
  REGION 1..5: note = source = /note="Description of Artificial Sequence: Synthetic peptide"
RNYMS

SEQ ID NO: 288 - protein, 16 aa, synthetic construct
  REGION 1..16: note = source = /note="Description of Artificial Sequence: Synthetic peptide"
GIYGGGRTYYAESVKG

SEQ ID NO: 289 - protein, 13 aa, synthetic construct
  REGION 1..13: note = source = /note="Description of Artificial Sequence: Synthetic peptide"
EDEFWSGYSAGVD

SEQ ID NO: 290 - protein, 7 aa, synthetic construct
  REGION 1..7: note = source = /note="Description of Artificial Sequence: Synthetic peptide"
GFTVSRN

SEQ ID NO: 291 - protein, 5 aa, synthetic construct
  REGION 1..5: note = source = /note="Description of Artificial Sequence: Synthetic peptide"
YGGGR

SEQ ID NO: 292 - protein, 13 aa, synthetic construct
  REGION 1..13: note = source = /note="Description of Artificial Sequence: Synthetic peptide"
EDEFWSGYSAGVD

SEQ ID NO: 293 - protein, 121 aa, synthetic construct
  REGION 1..121: note = source = /note="Description of Artificial Sequence: Synthetic polypeptide"
EVQLLESGGGLVRPGGSLRVSCAASGFTVSRNYMSWVRQAPGKGLEWVSGIYGGGRTYYAESVKGRFTISRDYSKNTLFLQMNTLRVEDTALYFCAREDEFWSGYSAGVDWGQGTLVTVSS

SEQ ID NO: 294 - DNA, 363 bp, synthetic construct
  misc_feature 1..363: note = source = /note="Description of Artificial Sequence: Synthetic polynucleotide"
  source 1..363: mol_type = other DNA
gaggtgcagctgttggagtccgggggaggcttggtccggcctggggggtccctgagagtctcatgtgcagcctctggattcaccgtcagtcgcaattacatgagttgggtccgccaggctccggggaagggactggagtgggtctcagggatttacggtggtggtaggacttactacgcagagtccgtgaagggccgattcaccatctccagagactattccaagaacacactgtttcttcaaatgaacaccctgagagtcgaggacacggccctgtatttctgtgcgagagaagacgaattttggagtgggtattctgctggggtcgactggggccagggaaccctggtcactgtctcctca

SEQ ID NO: 295 - protein, 451 aa, synthetic construct
  REGION 1..451: note = source = /note="Description of Artificial Sequence: Synthetic polypeptide"
EVQLLESGGGLVRPGGSLRVSCAASGFTVSRNYMSWVRQAPGKGLEWVSGIYGGGRTYYAESVKGRFTISRDYSKNTLFLQMNTLRVEDTALYFCAREDEFWSGYSAGVDWGQGTLVTVSSASTKGPSVFPLAPSSKSTSGGTAALGCLVKDYFPEPVTVSWNSGALTSGVHTFPAVLQSSGLYSLSSVVTVPSSSLGTQTYICNVNHKPSNTKVDKRVEPKSCDKTHTCPPCPAPELLGGPSVFLFPPKPKDTLMISRTPEVTCVVVDVSHEDPEVKFNWYVDGVEVHNAKTKPREEQYNSTYRVVSVLTVLHQDWLNGKEYKCKVSNKALPAPIEKTISKAKGQPREPQVYTLPPSREEMTKNQVSLTCLVKGFYPSDIAVEWESNGQPENNYKTTPPVLDSDGSFFLYSKLTVDKSRWQQGNVFSCSVMHEALHNHYTQKSLSLSPGK

SEQ ID NO: 296 - DNA, 1353 bp, synthetic construct
  misc_feature 1..1353: note = source = /note="Description of Artificial Sequence: Synthetic polynucleotide"
  source 1..1353: mol_type = other DNA
gaggtgcagctgttggagtccgggggaggcttggtccggcctggggggtccctgagagtctcatgtgcagcctctggattcaccgtcagtcgcaattacatgagttgggtccgccaggctccggggaagggactggagtgggtctcagggatttacggtggtggtaggacttactacgcagagtccgtgaagggccgattcaccatctccagagactattccaagaacacactgtttcttcaaatgaacaccctgagagtcgaggacacggccctgtatttctgtgcgagagaagacgaattttggagtgggtattctgctggggtcgactggggccagggaaccctggtcactgtctcctcagctagcaccaagggcccatcggtcttccccctggcaccctcctccaagagcacctctgggggcacagcggccctgggctgcctggtcaaggactacttccccgaaccggtgacggtgtcgtggaactcaggcgccctgaccagcggcgtgcacaccttcccggctgtcctacagtcctcaggactctactccctcagcagcgtggtgaccgtgccctccagcagcttgggcacccagacctacatctgcaacgtgaatcacaagcccagcaacaccaaggtggacaagagagttgagcccaaatcttgtgacaaaactcacacatgcccaccgtgcccagcacctgaactcctggggggaccgtcagtcttcctcttccccccaaaacccaaggacaccctcatgatctcccggacccctgaggtcacatgcgtggtggtggacgtgagccacgaagaccctgaggtcaagttcaactggtacgtggacggcgtggaggtgcataatgccaagacaaagccgcgggaggagcagtacaacagcacgtaccgtgtggtcagcgtcctcaccgtcctgcaccaggactggctgaatggcaaggagtacaagtgcaaggtctccaacaaagccctcccagcccccatcgagaaaaccatctccaaagccaaagggcagccccgagaaccacaggtgtacaccctgcccccatcccgggaggagatgaccaagaaccaggtcagcctgacctgcctggtcaaaggcttctatcccagcgacatcgccgtggagtgggagagcaatgggcagccggagaacaactacaagaccacgcctcccgtgctggactccgacggctccttcttcctctacagcaagctcaccgtggacaagagcaggtggcagcaggggaacgtcttctcatgctccgtgatgcatgaggctctgcacaaccactacacgcagaagagcctctccctgtctccgggtaaa

SEQ ID NO: 297 - protein, 11 aa, synthetic construct
  REGION 1..11: note = source = /note="Description of Artificial Sequence: Synthetic peptide"
RASQSISSYLN

SEQ ID NO: 298 - protein, 7 aa, synthetic construct
  REGION 1..7: note = source = /note="Description of Artificial Sequence: Synthetic peptide"
AASTLQT

SEQ ID NO: 299 - protein, 9 aa, synthetic construct
  REGION 1..9: note = source = /note="Description of Artificial Sequence: Synthetic peptide"
QQSYNTPRT

SEQ ID NO: 300 - protein, 7 aa, synthetic construct
  REGION 1..7: note = source = /note="Description of Artificial Sequence: Synthetic peptide"
SQSISSY

SEQ ID NO: 301 - skipped

SEQ ID NO: 302 - protein, 6 aa, synthetic construct
  REGION 1..6: note = source = /note="Description of Artificial Sequence: Synthetic peptide"
SYNTPR

SEQ ID NO: 303 - protein, 107 aa, synthetic construct
  REGION 1..107: note = source = /note="Description of Artificial Sequence: Synthetic polypeptide"
DIQVTQSPSSLSASVGDRVTITCRASQSISSYLNWYQQEPGKAPKLLIYAASTLQTGVPSRFSGSGSGTDFTLTISSLQPEDFATYYCQQSYNTPRTFGQGTKVEIK

SEQ ID NO: 304 - DNA, 323 bp, synthetic construct
  misc_feature 1..323: note = source = /note="Description of Artificial Sequence: Synthetic polynucleotide"
  source 1..323: mol_type = other DNA
gacatccaggtgacccagtctccatcctccctgtctgcatctgtaggagacagagtcaccatcacttgccgggcaagtcagagcattagcagctatttaaattggtatcagcaggaaccagggaaagcccctaaactcctgatctacgctgcatccactttgcaaactggggtcccatcacggttcagtggtagtggatctgggacagatttcactctcaccatcagcagtctgcaacctgaagattttgcaacttattactgtcaacagagttacaatacccctcgaaccttcggccaagggaccaaggtggaaatcaaacg

SEQ ID NO: 305 - protein, 214 aa, synthetic construct
  REGION 1..214: note = source = /note="Description of Artificial Sequence: Synthetic polypeptide"
DIQVTQSPSSLSASVGDRVTITCRASQSISSYLNWYQQEPGKAPKLLIYAASTLQTGVPSRFSGSGSGTDFTLTISSLQPEDFATYYCQQSYNTPRTFGQGTKVEIKRTVAAPSVFIFPPSDEQLKSGTASVVCLLNNFYPREAKVQWKVDNALQSGNSQESVTEQDSKDSTYSLSSTLTLSKADYEKHKVYACEVTHQGLSSPVTKSFNRGEC

SEQ ID NO: 306 - DNA, 642 bp, synthetic construct
  misc_feature 1..642: note = source = /note="Description of Artificial Sequence: Synthetic polynucleotide"
  source 1..642: mol_type = other DNA
gacatccaggtgacccagtctccatcctccctgtctgcatctgtaggagacagagtcaccatcacttgccgggcaagtcagagcattagcagctatttaaattggtatcagcaggaaccagggaaagcccctaaactcctgatctacgctgcatccactttgcaaactggggtcccatcacggttcagtggtagtggatctgggacagatttcactctcaccatcagcagtctgcaacctgaagattttgcaacttattactgtcaacagagttacaatacccctcgaaccttcggccaagggaccaaggtggaaatcaaacgtacggtggctgcaccatctgtcttcatcttcccgccatctgatgagcagttgaaatctggaactgcctctgttgtgtgcctgctgaataacttctatccccgcgaggccaaagtacagtggaaggtggataacgccctccaatcgggtaactcccaggagagtgtcacagagcaggacagcaaggacagcacctacagcctcagcagcaccctgacgctgagcaaagcagactacgagaaacacaaagtctacgcctgcgaagtcacccatcagggcctgagctcgcccgtcacaaagagcttcaaccgcggagagtgt

SEQ ID NO: 307 - protein, 7 aa, synthetic construct
  REGION 1..7: note = source = /note="Description of Artificial Sequence: Synthetic peptide"
NGGYYWS

SEQ ID NO: 308 - protein, 16 aa, synthetic construct
  REGION 1..16: note = source = /note="Description of Artificial Sequence: Synthetic peptide"
CIHYSGGTYYNPSLKS

SEQ ID NO: 309 - protein, 14 aa, synthetic construct
  REGION 1..14: note = source = /note="Description of Artificial Sequence: Synthetic peptide"
ALIAAPGISDWFDP

SEQ ID NO: 310 - protein, 9 aa, synthetic construct
  REGION 1..9: note = source = /note="Description of Artificial Sequence: Synthetic peptide"
GGSISNGGY

SEQ ID NO: 311 - protein, 5 aa, synthetic construct
  REGION 1..5: note = source = /note="Description of Artificial Sequence: Synthetic peptide"
HYSGG

SEQ ID NO: 312 - protein, 14 aa, synthetic construct
  REGION 1..14: note = source = /note="Description of Artificial Sequence: Synthetic peptide"
ALIAAPGISDWFDP

SEQ ID NO: 313 - protein, 124 aa, synthetic construct
  REGION 1..124: note = source = /note="Description of Artificial Sequence: Synthetic polypeptide"
QVQLQESGPGLVKPSQTLSLTCTVSGGSISNGGYYWSWIRLHPGKGLEWIGCIHYSGGTYYNPSLKSRVTVSLDTSKNQFSLNLISVTAADTAIYFCARALIAAPGISDWFDPWGQGTLVTVSS

SEQ ID NO: 314 - protein, 454 aa, synthetic construct
  REGION 1..454: note = source = /note="Description of Artificial Sequence: Synthetic polypeptide"
QVQLQESGPGLVKPSQTLSLTCTVSGGSISNGGYYWSWIRLHPGKGLEWIGCIHYSGGTYYNPSLKSRVTVSLDTSKNQFSLNLISVTAADTAIYFCARALIAAPGISDWFDPWGQGTLVTVSSASTKGPSVFPLAPSSKSTSGGTAALGCLVKDYFPEPVTVSWNSGALTSGVHTFPAVLQSSGLYSLSSVVTVPSSSLGTQTYICNVNHKPSNTKVDKKVEPKSCDKTHTCPPCPAPELLGGPSVFLFPPKPKDTLMISRTPEVTCVVVDVSHEDPEVKFNWYVDGVEVHNAKTKPREEQYNSTYRVVSVLTVLHQDWLNGKEYKCKVSNKALPAPIEKTISKAKGQPREPQVYTLPPSREEMTKNQVSLTCLVKGFYPSDIAVEWESNGQPENNYKTTPPVLDSDGSFFLYSKLTVDKSRWQQGNVFSCSVMHEALHNHYTQKSLSLSPGK

SEQ ID NO: 315 - protein, 13 aa, synthetic construct
  REGION 1..13: note = source = /note="Description of Artificial Sequence: Synthetic peptide"
SGSNSNVGHNYVS

SEQ ID NO: 316 - protein, 7 aa, synthetic construct
  REGION 1..7: note = source = /note="Description of Artificial Sequence: Synthetic peptide"
DNNKRPS

SEQ ID NO: 317 - protein, 11 aa, synthetic construct
  REGION 1..11: note = source = /note="Description of Artificial Sequence: Synthetic peptide"
GTWDSSLSAGV

SEQ ID NO: 318 - protein, 9 aa, synthetic construct
  REGION 1..9: note = source = /note="Description of Artificial Sequence: Synthetic peptide"
SNSNVGHNY

SEQ ID NO: 319 - skipped

SEQ ID NO: 320 - protein, 8 aa, synthetic construct
  REGION 1..8: note = source = /note="Description of Artificial Sequence: Synthetic peptide"
WDSSLSAG

SEQ ID NO: 321 - protein, 110 aa, synthetic construct
  REGION 1..110: note = source = /note="Description of Artificial Sequence: Synthetic polypeptide"
QSVLTQPPSVSAAPGQKVTISCSGSNSNVGHNYVSWYQQLPGTAPKLLIYDNNKRPSGIPDRFSGSKSGTSATLGITGLQTGDEADYYCGTWDSSLSAGVFGGGTKVTVL

SEQ ID NO: 322 - protein, 216 aa, synthetic construct
  REGION 1..216: note = source = /note="Description of Artificial Sequence: Synthetic polypeptide"
QSVLTQPPSVSAAPGQKVTISCSGSNSNVGHNYVSWYQQLPGTAPKLLIYDNNKRPSGIPDRFSGSKSGTSATLGITGLQTGDEADYYCGTWDSSLSAGVFGGGTKVTVLGQPKAAPSVTLFPPSSEELQANKATLVCLISDFYPGAVTVAWKADSSPVKAGVETTTPSKQSNNKYAASSYLSLTPEQWKSHRSYSCQVTHEGSTVEKTVAPTECS

SEQ ID NO: 323 - protein, 5 aa, synthetic construct
  REGION 1..5: note = source = /note="Description of Artificial Sequence: Synthetic peptide"
SSWMN

SEQ ID NO: 324 - protein, 17 aa, synthetic construct
  REGION 1..17: note = source = /note="Description of Artificial Sequence: Synthetic peptide"
RIYPGDADTYYSGKFKG

SEQ ID NO: 325 - protein, 7 aa, synthetic construct
  REGION 1..7: note = source = /note="Description of Artificial Sequence: Synthetic peptide"
HSSGFTY

SEQ ID NO: 326 - protein, 7 aa, synthetic construct
  REGION 1..7: note = source = /note="Description of Artificial Sequence: Synthetic peptide"
GYTFSSS

SEQ ID NO: 327 - protein, 6 aa, synthetic construct
  REGION 1..6: note = source = /note="Description of Artificial Sequence: Synthetic peptide"
YPGDAD

SEQ ID NO: 328 - protein, 7 aa, synthetic construct
  REGION 1..7: note = source = /note="Description of Artificial Sequence: Synthetic peptide"
HSSGFTY

SEQ ID NO: 329 - protein, 116 aa, synthetic construct
  REGION 1..116: note = source = /note="Description of Artificial Sequence: Synthetic polypeptide"
QVQLVQSGAEVKKPGASVKVSCKASGYTFSSSWMNWVRQAPGQRLEWMGRIYPGDADTYYSGKFKGRVTITADSSARTAYMELSSLRSEDTAVYYCAIHSSGFTYWGQGTLVTVSS

SEQ ID NO: 330 - DNA, 350 bp, synthetic construct
  misc_feature 1..350: note = source = /note="Description of Artificial Sequence: Synthetic polynucleotide"
  source 1..350: mol_type = other DNA
caggtccagcttgtgcagtctggggctgaggtgaagaagcctggggcctcagtgaaggtttcctgcaaggcttctggctatacattcagcagctcttggatgaactgggtgcgccaggcccccggacaaaggcttgagtggatgggacggatctatccaggagacgccgatacttactacagtgggaaattcaagggcagagtcaccattaccgccgacagctccgcgagaacagcctacatggagctgagcagcctgagatctgaagacacggctgtgtattactgtgcgatccacagctcgggctttacttactggggccagggcaccctggtcaccgtctcctcagc

SEQ ID NO: 331 - protein, 446 aa, synthetic construct
  REGION 1..446: note = source = /note="Description of Artificial Sequence: Synthetic polypeptide"
QVQLVQSGAEVKKPGASVKVSCKASGYTFSSSWMNWVRQAPGQRLEWMGRIYPGDADTYYSGKFKGRVTITADSSARTAYMELSSLRSEDTAVYYCAIHSSGFTYWGQGTLVTVSSASTKGPSVFPLAPSSKSTSGGTAALGCLVKDYFPEPVTVSWNSGALTSGVHTFPAVLQSSGLYSLSSVVTVPSSSLGTQTYICNVNHKPSNTKVDKRVEPKSCDKTHTCPPCPAPELLGGPSVFLFPPKPKDTLMISRTPEVTCVVVDVSHEDPEVKFNWYVDGVEVHNAKTKPREEQYNSTYRVVSVLTVLHQDWLNGKEYKCKVSNKALPAPIEKTISKAKGQPREPQVYTLPPSREEMTKNQVSLTCLVKGFYPSDIAVEWESNGQPENNYKTTPPVLDSDGSFFLYSKLTVDKSRWQQGNVFSCSVMHEALHNHYTQKSLSLSPGK

SEQ ID NO: 332 - DNA, 1338 bp, synthetic construct
  misc_feature 1..1338: note = source = /note="Description of Artificial Sequence: Synthetic polynucleotide"
  source 1..1338: mol_type = other DNA
caggtccagcttgtgcagtctggggctgaggtgaagaagcctggggcctcagtgaaggtttcctgcaaggcttctggctatacattcagcagctcttggatgaactgggtgcgccaggcccccggacaaaggcttgagtggatgggacggatctatccaggagacgccgatacttactacagtgggaaattcaagggcagagtcaccattaccgccgacagctccgcgagaacagcctacatggagctgagcagcctgagatctgaagacacggctgtgtattactgtgcgatccacagctcgggctttacttactggggccagggcaccctggtcaccgtctcctcagctagcaccaagggcccatcggtcttccccctggcaccctcctccaagagcacctctgggggcacagcggccctgggctgcctggtcaaggactacttccccgaaccggtgacggtgtcgtggaactcaggcgccctgaccagcggcgtgcacaccttcccggctgtcctacagtcctcaggactctactccctcagcagcgtggtgaccgtgccctccagcagcttgggcacccagacctacatctgcaacgtgaatcacaagcccagcaacaccaaggtggacaagagagttgagcccaaatcttgtgacaaaactcacacatgcccaccgtgcccagcacctgaactcctggggggaccgtcagtcttcctcttccccccaaaacccaaggacaccctcatgatctcccggacccctgaggtcacatgcgtggtggtggacgtgagccacgaagaccctgaggtcaagttcaactggtacgtggacggcgtggaggtgcataatgccaagacaaagccgcgggaggagcagtacaacagcacgtaccgtgtggtcagcgtcctcaccgtcctgcaccaggactggctgaatggcaaggagtacaagtgcaaggtctccaacaaagccctcccagcccccatcgagaaaaccatctccaaagccaaagggcagccccgagaaccacaggtgtacaccctgcccccatcccgggaggagatgaccaagaaccaggtcagcctgacctgcctggtcaaaggcttctatcccagcgacatcgccgtggagtgggagagcaatgggcagccggagaacaactacaagaccacgcctcccgtgctggactccgacggctccttcttcctctacagcaagctcaccgtggacaagagcaggtggcagcaggggaacgtcttctcatgctccgtgatgcatgaggctctgcacaaccactacacgcagaagagcctctccctgtctccgggtaaa

SEQ ID NO: 333 - protein, 11 aa, synthetic construct
  REGION 1..11: note = source = /note="Description of Artificial Sequence: Synthetic peptide"
RASQDISDYLN

SEQ ID NO: 334 - protein, 7 aa, synthetic construct
  REGION 1..7: note = source = /note="Description of Artificial Sequence: Synthetic peptide"
YTSRLHS

SEQ ID NO: 335 - protein, 9 aa, synthetic construct
  REGION 1..9: note = source = /note="Description of Artificial Sequence: Synthetic peptide"
QQTHTLPFT

SEQ ID NO: 336 - protein, 7 aa, synthetic construct
  REGION 1..7: note = source = /note="Description of Artificial Sequence: Synthetic peptide"
SQDISDY

SEQ ID NO: 337 - skipped

SEQ ID NO: 338 - protein, 6 aa, synthetic construct
  REGION 1..6: note = source = /note="Description of Artificial Sequence: Synthetic peptide"
THTLPF

SEQ ID NO: 339 - protein, 107 aa, synthetic construct
  REGION 1..107: note = source = /note="Description of Artificial Sequence: Synthetic polypeptide"
DIQMTQSPSSLSASVGDRVTITCRASQDISDYLNWYQQKPGKAPKLLIYYTSRLHSGVPSRFSGSGSGTDYTLTISSLQPEDFATYFCQQTHTLPFTFGGGTKVEIK

SEQ ID NO: 340 - DNA, 323 bp, synthetic construct
  misc_feature 1..323: note = source = /note="Description of Artificial Sequence: Synthetic polynucleotide"
  source 1..323: mol_type = other DNA
gacatccagatgacccagtctccatcctccctgtctgcatctgtaggagacagagtcaccatcacttgcagggcaagtcaggacattagcgattatttaaactggtatcagcagaaaccagggaaagcccctaagctcctgatctattatacatcaagattacactcaggggtcccatcaaggttcagtggcagtggatctgggacagattacactctcaccatcagcagtctgcaacctgaagattttgcaacttacttctgtcaacagactcatacgcttcctttcacgttcggcggagggaccaaggtggagatcaaacg

SEQ ID NO: 341 - protein, 214 aa, synthetic construct
  REGION 1..214: note = source = /note="Description of Artificial Sequence: Synthetic polypeptide"
DIQMTQSPSSLSASVGDRVTITCRASQDISDYLNWYQQKPGKAPKLLIYYTSRLHSGVPSRFSGSGSGTDYTLTISSLQPEDFATYFCQQTHTLPFTFGGGTKVEIKRTVAAPSVFIFPPSDEQLKSGTASVVCLLNNFYPREAKVQWKVDNALQSGNSQESVTEQDSKDSTYSLSSTLTLSKADYEKHKVYACEVTHQGLSSPVTKSFNRGEC

SEQ ID NO: 342 - DNA, 642 bp, synthetic construct
  misc_feature 1..642: note = source = /note="Description of Artificial Sequence: Synthetic polynucleotide"
  source 1..642: mol_type = other DNA
gacatccagatgacccagtctccatcctccctgtctgcatctgtaggagacagagtcaccatcacttgcagggcaagtcaggacattagcgattatttaaactggtatcagcagaaaccagggaaagcccctaagctcctgatctattatacatcaagattacactcaggggtcccatcaaggttcagtggcagtggatctgggacagattacactctcaccatcagcagtctgcaacctgaagattttgcaacttacttctgtcaacagactcatacgcttcctttcacgttcggcggagggaccaaggtggagatcaaacgtacggtggctgcaccatctgtcttcatcttcccgccatctgatgagcagttgaaatctggaactgcctctgttgtgtgcctgctgaataacttctatccccgcgaggccaaagtacagtggaaggtggataacgccctccaatcgggtaactcccaggagagtgtcacagagcaggacagcaaggacagcacctacagcctcagcagcaccctgacgctgagcaaagcagactacgagaaacacaaagtctacgcctgcgaagtcacccatcagggcctgagctcgcccgtcacaaagagcttcaaccgcggagagtgt

SEQ ID NO: 343 - protein, 5 aa, synthetic construct
  REGION 1..5: note = source = /note="Description of Artificial Sequence: Synthetic peptide"
NYWMH

SEQ ID NO: 344 - protein, 17 aa, synthetic construct
  REGION 1..17: note = source = /note="Description of Artificial Sequence: Synthetic peptide"
NIYPGSGNTNYGENFKS

SEQ ID NO: 345 - protein, 16 aa, synthetic construct
  REGION 1..16: note = source = /note="Description of Artificial Sequence: Synthetic peptide"
SAIYYGYDGHYFAMDY

SEQ ID NO: 346 - protein, 7 aa, synthetic construct
  REGION 1..7: note = source = /note="Description of Artificial Sequence: Synthetic peptide"
GYTFTNY

SEQ ID NO: 347 - protein, 6 aa, synthetic construct
  REGION 1..6: note = source = /note="Description of Artificial Sequence: Synthetic peptide"
YPGSGN

SEQ ID NO: 348 - protein, 16 aa, synthetic construct
  REGION 1..16: note = source = /note="Description of Artificial Sequence: Synthetic peptide"
SAIYYGYDGHYFAMDY

SEQ ID NO: 349 - protein, 125 aa, synthetic construct
  REGION 1..125: note = source = /note="Description of Artificial Sequence: Synthetic polypeptide"
QVQLQQPGSELVRPGASVKLSCKASGYTFTNYWMHWVKQGHGQGLEWIGNIYPGSGNTNYGENFKSKGTLTVDTSSSTAYMHLSRLTSEDSAVYYCSRSAIYYGYDGHYFAMDYWGQGTSVTVSS

SEQ ID NO: 350 - protein, 11 aa, synthetic construct
  REGION 1..11: note = source = /note="Description of Artificial Sequence: Synthetic peptide"
KASQDIRKYIA

SEQ ID NO: 351 - protein, 7 aa, synthetic construct
  REGION 1..7: note = source = /note="Description of Artificial Sequence: Synthetic peptide"
YTSTLQS

SEQ ID NO: 352 - protein, 9 aa, synthetic construct
  REGION 1..9: note = source = /note="Description of Artificial Sequence: Synthetic peptide"
LQYDNILFT

SEQ ID NO: 353 - protein, 7 aa, synthetic construct
  REGION 1..7: note = source = /note="Description of Artificial Sequence: Synthetic peptide"
SQDIRKY

SEQ ID NO: 354 - skipped

SEQ ID NO: 355 - protein, 6 aa, synthetic construct
  REGION 1..6: note = source = /note="Description of Artificial Sequence: Synthetic peptide"
YDNILF

SEQ ID NO: 356 - protein, 107 aa, synthetic construct
  REGION 1..107: note = source = /note="Description of Artificial Sequence: Synthetic polypeptide"
DIQMTQSPSSLSASLGGKVTITCKASQDIRKYIAWYQHKPGKGPRLLINYTSTLQSGIPSRFRGSGSGRDYSFSISNLEPEDIATYYCLQYDNILFTFGTGTKLEIK

SEQ ID NO: 357 - protein, 5 aa, synthetic construct
  REGION 1..5: note = source = /note="Description of Artificial Sequence: Synthetic peptide"
SCWMN

SEQ ID NO: 358 - protein, 17 aa, synthetic construct
  REGION 1..17: note = source = /note="Description of Artificial Sequence: Synthetic peptide"
RIYPGDGDTKYTEKFKD

SEQ ID NO: 359 - protein, 7 aa, synthetic construct
  REGION 1..7: note = source = /note="Description of Artificial Sequence: Synthetic peptide"
SGSGLPY

SEQ ID NO: 360 - protein, 7 aa, synthetic construct
  REGION 1..7: note = source = /note="Description of Artificial Sequence: Synthetic peptide"
GYSFSSC

SEQ ID NO: 361 - protein, 6 aa, synthetic construct
  REGION 1..6: note = source = /note="Description of Artificial Sequence: Synthetic peptide"
YPGDGD

SEQ ID NO: 362 - protein, 7 aa, synthetic construct
  REGION 1..7: note = source = /note="Description of Artificial Sequence: Synthetic peptide"
SGSGLPY

SEQ ID NO: 363 - protein, 116 aa, synthetic construct
  REGION 1..116: note = source = /note="Description of Artificial Sequence: Synthetic polypeptide"
QVHLQQSGPELVKPGASVTISCKTSGYSFSSCWMNWVKQRPGQGLEWIGRIYPGDGDTKYTEKFKDKATLTADKSSSTAYMQLSSLTSVDSALYFCAISGSGLPYWGQGTLVTVSE

SEQ ID NO: 364 - protein, 11 aa, synthetic construct
  REGION 1..11: note = source = /note="Description of Artificial Sequence: Synthetic peptide"
RASQDIHNYLN

SEQ ID NO: 365 - protein, 7 aa, synthetic construct
  REGION 1..7: note = source = /note="Description of Artificial Sequence: Synthetic peptide"
STSRLHS

SEQ ID NO: 366 - protein, 9 aa, synthetic construct
  REGION 1..9: note = source = /note="Description of Artificial Sequence: Synthetic peptide"
QQTHTLPLT

SEQ ID NO: 367 - protein, 7 aa, synthetic construct
  REGION 1..7: note = source = /note="Description of Artificial Sequence: Synthetic peptide"
SQDIHNY

SEQ ID NO: 368 - skipped

SEQ ID NO: 369 - protein, 6 aa, synthetic construct
  REGION 1..6: note = source = /note="Description of Artificial Sequence: Synthetic peptide"
THTLPL

SEQ ID NO: 370 - protein, 107 aa, synthetic construct
  REGION 1..107: note = source = /note="Description of Artificial Sequence: Synthetic polypeptide"
DIQMTQTTSSLSASLGDRVTISCRASQDIHNYLNWYQQKPDGTIKLLIYSTSRLHSGVPSRFSGSGSGTHYSLTINNLEQEDIATYFCQQTHTLPLTFGAGTKLELK

SEQ ID NO: 371 - protein, 5 aa, synthetic construct
  REGION 1..5: note = source = /note="Description of Artificial Sequence: Synthetic peptide"
SYWMN

SEQ ID NO: 372 - protein, 17 aa, synthetic construct
  REGION 1..17: note = source = /note="Description of Artificial Sequence: Synthetic peptide"
QIYPGNGDTNYNGKFKG

SEQ ID NO: 373 - protein, 12 aa, synthetic construct
  REGION 1..12: note = source = /note="Description of Artificial Sequence: Synthetic peptide"
EARQGYHYAMDY

SEQ ID NO: 374 - protein, 7 aa, synthetic construct
  REGION 1..7: note = source = /note="Description of Artificial Sequence: Synthetic peptide"
GYAFSSY

SEQ ID NO: 375 - protein, 6 aa, synthetic construct
  REGION 1..6: note = source = /note="Description of Artificial Sequence: Synthetic peptide"
YPGNGD

SEQ ID NO: 376 - protein, 12 aa, synthetic construct
  REGION 1..12: note = source = /note="Description of Artificial Sequence: Synthetic peptide"
EARQGYHYAMDY

SEQ ID NO: 377 - protein, 121 aa, synthetic construct
  REGION 1..121: note = source = /note="Description of Artificial Sequence: Synthetic polypeptide"
QVQLQQSGAGLVRPGSSVKISCKTSGYAFSSYWMNWVKQRPGQGLEWIGQIYPGNGDTNYNGKFKGKATLTADKSSNTAYIQLNSLTSEDSAVYFCAREARQGYHYAMDYWGQGTSVTVSL

SEQ ID NO: 378 - protein, 12 aa, synthetic construct
  REGION 1..12: note = source = /note="Description of Artificial Sequence: Synthetic peptide"
SASSMINSNYLH

SEQ ID NO: 379 - protein, 7 aa, synthetic construct
  REGION 1..7: note = source = /note="Description of Artificial Sequence: Synthetic peptide"
RTSNLAS

SEQ ID NO: 380 - protein, 8 aa, synthetic construct
  REGION 1..8: note = source = /note="Description of Artificial Sequence: Synthetic peptide"
QQGSNIFT

SEQ ID NO: 381 - protein, 8 aa, synthetic construct
  REGION 1..8: note = source = /note="Description of Artificial Sequence: Synthetic peptide"
SSMINSNY

SEQ ID NO: 382 - skipped

SEQ ID NO: 383 - protein, 5 aa, synthetic construct
  REGION 1..5: note = source = /note="Description of Artificial Sequence: Synthetic peptide"
GSNIF

SEQ ID NO: 384 - protein, 107 aa, synthetic construct
  REGION 1..107: note = source = /note="Description of Artificial Sequence: Synthetic polypeptide"
EIVFTQSPTTMAAFPGEKITITCSASSMINSNYLHWYQQKPGFSPKVLIYRTSNLASGVPARFSGTGSGTSFSLTIGTMEAEDVATYYCQQGSNIFTFGSGTKLEIK

SEQ ID NO: 385 - protein, 5 aa, synthetic construct
  REGION 1..5: note = source = /note="Description of Artificial Sequence: Synthetic peptide"
NSWMN

SEQ ID NO: 386 - protein, 17 aa, synthetic construct
  REGION 1..17: note = source = /note="Description of Artificial Sequence: Synthetic peptide"
RIYPGDGDTQYNEKFKG

SEQ ID NO: 387 - protein, 7 aa, synthetic construct
  REGION 1..7: note = source = /note="Description of Artificial Sequence: Synthetic peptide"
SRSGLDY

SEQ ID NO: 388 - protein, 7 aa, synthetic construct
  REGION 1..7: note = source = /note="Description of Artificial Sequence: Synthetic peptide"
GFTFSNS

SEQ ID NO: 389 - protein, 6 aa, synthetic construct
  REGION 1..6: note = source = /note="Description of Artificial Sequence: Synthetic peptide"
YPGDGD

SEQ ID NO: 390 - protein, 7 aa, synthetic construct
  REGION 1..7: note = source = /note="Description of Artificial Sequence: Synthetic peptide"
SRSGLDY

SEQ ID NO: 391 - protein, 116 aa, synthetic construct
  REGION 1..116: note = source = /note="Description of Artificial Sequence: Synthetic polypeptide"
QVQLQQSGPELVKPGASVRISCKVSGFTFSNSWMNWVKQRPGQGLEWIGRIYPGDGDTQYNEKFKGKATLTADTSSNTAYIQLNSLTSVDSAVFFCARSRSGLDYWGQGTTLTVSS

SEQ ID NO: 392 - protein, 11 aa, synthetic construct
  REGION 1..11: note = source = /note="Description of Artificial Sequence: Synthetic peptide"
RASQDIYNYLN

SEQ ID NO: 393 - protein, 7 aa, synthetic construct
  REGION 1..7: note = source = /note="Description of Artificial Sequence: Synthetic peptide"
STSRLHS

SEQ ID NO: 394 - protein, 9 aa, synthetic construct
  REGION 1..9: note = source = /note="Description of Artificial Sequence: Synthetic peptide"
HQSHTVPFT

SEQ ID NO: 395 - protein, 7 aa, synthetic construct
  REGION 1..7: note = source = /note="Description of Artificial Sequence: Synthetic peptide"
SQDIYNY

SEQ ID NO: 396 - skipped

SEQ ID NO: 397 - protein, 6 aa, synthetic construct
  REGION 1..6: note = source = /note="Description of Artificial Sequence: Synthetic peptide"
SHTVPF

SEQ ID NO: 398 - protein, 107 aa, synthetic construct
  REGION 1..107: note = source = /note="Description of Artificial Sequence: Synthetic polypeptide"
DIQMTQSTSSLSASLGDRVTISCRASQDIYNYLNWFQQKPDGTVKPLIYSTSRLHSGVSSRFSGSGSGTDYSLTISNLEREDIATYFCHQSHTVPFTFGSGTKLEIK

SEQ ID NO: 399 - protein, 5 aa, synthetic construct
  REGION 1..5: note = source = /note="Description of Artificial Sequence: Synthetic peptide"
SSWIN

SEQ ID NO: 400 - protein, 17 aa, synthetic construct
  REGION 1..17: note = source = /note="Description of Artificial Sequence: Synthetic peptide"
RIYPGDGDTNYNGKFKG

SEQ ID NO: 401 - protein, 7 aa, synthetic construct
  REGION 1..7: note = source = /note="Description of Artificial Sequence: Synthetic peptide"
HSSGFPH

SEQ ID NO: 402 - protein, 7 aa, synthetic construct
  REGION 1..7: note = source = /note="Description of Artificial Sequence: Synthetic peptide"
GYTFSSS

SEQ ID NO: 403 - protein, 6 aa, synthetic construct
  REGION 1..6: note = source = /note="Description of Artificial Sequence: Synthetic peptide"
YPGDGD

SEQ ID NO: 404 - protein, 7 aa, synthetic construct
  REGION 1..7: note = source = /note="Description of Artificial Sequence: Synthetic peptide"
HSSGFPH

SEQ ID NO: 405 - protein, 116 aa, synthetic construct
  REGION 1..116: note = source = /note="Description of Artificial Sequence: Synthetic polypeptide"
QVQLQQSGPELVKPGASVKISCKASGYTFSSSWINWVKQRPGQGLEWIGRIYPGDGDTNYNGKFKGKATLTADKSSSTVDMHLSSLTYVDSAVYFCAIHSSGFPHWGQGTLVTVSA

SEQ ID NO: 406 - protein, 11 aa, synthetic construct
  REGION 1..11: note = source = /note="Description of Artificial Sequence: Synthetic peptide"
RTSQDISDYLN

SEQ ID NO: 407 - protein, 7 aa, synthetic construct
  REGION 1..7: note = source = /note="Description of Artificial Sequence: Synthetic peptide"
YTSRLHS

SEQ ID NO: 408 - protein, 9 aa, synthetic construct
  REGION 1..9: note = source = /note="Description of Artificial Sequence: Synthetic peptide"
QQTNTLPFT

SEQ ID NO: 409 - protein, 7 aa, synthetic construct
  REGION 1..7: note = source = /note="Description of Artificial Sequence: Synthetic peptide"
SQDISDY

SEQ ID NO: 410 - skipped

SEQ ID NO: 411 - protein, 6 aa, synthetic construct
  REGION 1..6: note = source = /note="Description of Artificial Sequence: Synthetic peptide"
TNTLPF

SEQ ID NO: 412 - protein, 107 aa, synthetic construct
  REGION 1..107: note = source = /note="Description of Artificial Sequence: Synthetic polypeptide"
DIQMTQTTSSLSASLGGRVTISCRTSQDISDYLNWYQQKPDGAVKLLIYYTSRLHSGVPSRFSGSGSGTDYSLTISNLEQEDIATYFCQQTNTLPFTFGGGTKLEIK

SEQ ID NO: 413 - protein, 5 aa, synthetic construct
  REGION 1..5: note = source = /note="Description of Artificial Sequence: Synthetic peptide"
RYWMN

SEQ ID NO: 414 - protein, 17 aa, synthetic construct
  REGION 1..17: note = source = /note="Description of Artificial Sequence: Synthetic peptide"
QIYPGDGDTKYNGKFKD

SEQ ID NO: 415 - protein, 8 aa, synthetic construct
  REGION 1..8: note = source = /note="Description of Artificial Sequence: Synthetic peptide"
YGNYGMDY

SEQ ID NO: 416 - protein, 7 aa, synthetic construct
  REGION 1..7: note = source = /note="Description of Artificial Sequence: Synthetic peptide"
GYAFSRY

SEQ ID NO: 417 - protein, 6 aa, synthetic construct
  REGION 1..6: note = source = /note="Description of Artificial Sequence: Synthetic peptide"
YPGDGD

SEQ ID NO: 418 - protein, 8 aa, synthetic construct
  REGION 1..8: note = source = /note="Description of Artificial Sequence: Synthetic peptide"
YGNYGMDY

SEQ ID NO: 419 - protein, 117 aa, synthetic construct
  REGION 1..117: note = source = /note="Description of Artificial Sequence: Synthetic polypeptide"
QVQLQQSGAELVRPGSSVKISCKASGYAFSRYWMNWVKQRPGQGLEWIGQIYPGDGDTKYNGKFKDTATLTADKSSSTAYLQLSSLTSEDSAVYFCAKYGNYGMDYWGQGTSVTVSS

SEQ ID NO: 420 - protein, 16 aa, synthetic construct
  REGION 1..16: note = source = /note="Description of Artificial Sequence: Synthetic peptide"
RSSQSLEYGNGNTYLN

SEQ ID NO: 421 - protein, 7 aa, synthetic construct
  REGION 1..7: note = source = /note="Description of Artificial Sequence: Synthetic peptide"
RVSNRFS

SEQ ID NO: 422 - protein, 9 aa, synthetic construct
  REGION 1..9: note = source = /note="Description of Artificial Sequence: Synthetic peptide"
LQFTHVPYT

SEQ ID NO: 423 - protein, 12 aa, synthetic construct
  REGION 1..12: note = source = /note="Description of Artificial Sequence: Synthetic peptide"
SQSLEYGNGNTY

SEQ ID NO: 424 - skipped

SEQ ID NO: 425 - protein, 6 aa, synthetic construct
  REGION 1..6: note = source = /note="Description of Artificial Sequence: Synthetic peptide"
FTHVPY

SEQ ID NO: 426 - protein, 112 aa, synthetic construct
  REGION 1..112: note = source = /note="Description of Artificial Sequence: Synthetic polypeptide"
DAVMTQTPLSLPVSLGDQASISCRSSQSLEYGNGNTYLNWYLQKPGQSPQLLIYRVSNRFSGVLDRFSGSGSGTDFTLKISRVEAEDLGVYFCLQFTHVPYTFGGGTKLEIK

SEQ ID NO: 427 - protein, 5 aa, synthetic construct
  REGION 1..5: note = source = /note="Description of Artificial Sequence: Synthetic peptide"
GYTMN

SEQ ID NO: 428 - protein, 17 aa, synthetic construct
  REGION 1..17: note = source = /note="Description of Artificial Sequence: Synthetic peptide"
LFNPYNGGTRYNQKFKG

SEQ ID NO: 429 - protein, 13 aa, synthetic construct
  REGION 1..13: note = source = /note="Description of Artificial Sequence: Synthetic peptide"
LRNYGIGDDFFDY

SEQ ID NO: 430 - protein, 7 aa, synthetic construct
  REGION 1..7: note = source = /note="Description of Artificial Sequence: Synthetic peptide"
GYSFTGY

SEQ ID NO: 431 - protein, 6 aa, synthetic construct
  REGION 1..6: note = source = /note="Description of Artificial Sequence: Synthetic peptide"
NPYNGG

SEQ ID NO: 432 - protein, 13 aa, synthetic construct
  REGION 1..13: note = source = /note="Description of Artificial Sequence: Synthetic peptide"
LRNYGIGDDFFDY

SEQ ID NO: 433 - protein, 122 aa, synthetic construct
  REGION 1..122: note = source = /note="Description of Artificial Sequence: Synthetic polypeptide"
EVQLQQSGPELVKPGASMKISCKASGYSFTGYTMNWVKQSHGENLEWIGLFNPYNGGTRYNQKFKGKATLTVDKSSSTAYMELLSLTSEDSAVYYCARLRNYGIGDDFFDYWGQGTTLTVSS

SEQ ID NO: 434 - protein, 11 aa, synthetic construct
  REGION 1..11: note = source = /note="Description of Artificial Sequence: Synthetic peptide"
KASQDVGTAVA

SEQ ID NO: 435 - protein, 7 aa, synthetic construct
  REGION 1..7: note = source = /note="Description of Artificial Sequence: Synthetic peptide"
WASTRHT

SEQ ID NO: 436 - protein, 9 aa, synthetic construct
  REGION 1..9: note = source = /note="Description of Artificial Sequence: Synthetic peptide"
QQYSNYPYT

SEQ ID NO: 437 - protein, 7 aa, synthetic construct
  REGION 1..7: note = source = /note="Description of Artificial Sequence: Synthetic peptide"
SQDVGTA

SEQ ID NO: 438 - skipped

SEQ ID NO: 439 - protein, 6 aa, synthetic construct
  REGION 1..6: note = source = /note="Description of Artificial Sequence: Synthetic peptide"
YSNYPY

SEQ ID NO: 440 - protein, 107 aa, synthetic construct
  REGION 1..107: note = source = /note="Description of Artificial Sequence: Synthetic polypeptide"
DIVMTQSHKFMSTSVGDRVSITCKASQDVGTAVAWYQQKPGQSPKLLIYWASTRHTGVPDRFTGSGSGTDFTLTISNVQSEDLTDYFCQQYSNYPYTFGGGTKLEIK

SEQ ID NO: 441 - protein, 5 aa, synthetic construct
  REGION 1..5: note = source = /note="Description of Artificial Sequence: Synthetic peptide"
GYTMN

SEQ ID NO: 442 - protein, 17 aa, synthetic construct
  REGION 1..17: note = source = /note="Description of Artificial Sequence: Synthetic peptide"
LFNPYNGGINYNQKFKG

SEQ ID NO: 443 - protein, 13 aa, synthetic construct
  REGION 1..13: note = source = /note="Description of Artificial Sequence: Synthetic peptide"
LRYYGIGDDFFDY

SEQ ID NO: 444 - protein, 7 aa, synthetic construct
  REGION 1..7: note = source = /note="Description of Artificial Sequence: Synthetic peptide"
GYSFTGY

SEQ ID NO: 445 - protein, 6 aa, synthetic construct
  REGION 1..6: note = source = /note="Description of Artificial Sequence: Synthetic peptide"
NPYNGG

SEQ ID NO: 446 - protein, 13 aa, synthetic construct
  REGION 1..13: note = source = /note="Description of Artificial Sequence: Synthetic peptide"
LRYYGIGDDFFDY

SEQ ID NO: 447 - protein, 122 aa, synthetic construct
  REGION 1..122: note = source = /note="Description of Artificial Sequence: Synthetic polypeptide"
EVQLQQSGPELVKPGASMKISCKASGYSFTGYTMNWVKQSHGKNLEWIGLFNPYNGGINYNQKFKGKATLTVDKSSSTAYMELLSLTSEDSAVYYCARLRYYGIGDDFFDYWGQGTSLTVSS

SEQ ID NO: 448 - protein, 11 aa, synthetic construct
  REGION 1..11: note = source = /note="Description of Artificial Sequence: Synthetic peptide"
KASRDVGTAVA

SEQ ID NO: 449 - protein, 7 aa, synthetic construct
  REGION 1..7: note = source = /note="Description of Artificial Sequence: Synthetic peptide"
WASTRHT

SEQ ID NO: 450 - protein, 9 aa, synthetic construct
  REGION 1..9: note = source = /note="Description of Artificial Sequence: Synthetic peptide"
QQYSNYPYT

SEQ ID NO: 451 - protein, 7 aa, synthetic construct
  REGION 1..7: note = source = /note="Description of Artificial Sequence: Synthetic peptide"
SRDVGTA

SEQ ID NO: 452 - skipped

SEQ ID NO: 453 - protein, 6 aa, synthetic construct
  REGION 1..6: note = source = /note="Description of Artificial Sequence: Synthetic peptide"
YSNYPY

SEQ ID NO: 454 - protein, 107 aa, synthetic construct
  REGION 1..107: note = source = /note="Description of Artificial Sequence: Synthetic polypeptide"
DIVMTQSHKFMSTSVGDRVSITCKASRDVGTAVAWYQQKPGQSPKLLIYWASTRHTGVPDRFTGSGSGTDFTLTISNVQSEDLADYFCQQYSNYPYTFGGGTKLEMK

SEQ ID NO: 455 - protein, 5 aa, synthetic construct
  REGION 1..5: note = source = /note="Description of Artificial Sequence: Synthetic peptide"
GYTMN

SEQ ID NO: 456 - protein, 17 aa, synthetic construct
  REGION 1..17: note = source = /note="Description of Artificial Sequence: Synthetic peptide"
LFNPYNGGPNYNQKFKG

SEQ ID NO: 457 - protein, 13 aa, synthetic construct
  REGION 1..13: note = source = /note="Description of Artificial Sequence: Synthetic peptide"
LRYYGIGDDFFDY

SEQ ID NO: 458 - protein, 7 aa, synthetic construct
  REGION 1..7: note = source = /note="Description of Artificial Sequence: Synthetic peptide"
GYSFTGY

SEQ ID NO: 459 - protein, 6 aa, synthetic construct
  REGION 1..6: note = source = /note="Description of Artificial Sequence: Synthetic peptide"
NPYNGG

SEQ ID NO: 460 - protein, 13 aa, synthetic construct
  REGION 1..13: note = source = /note="Description of Artificial Sequence: Synthetic peptide"
LRYYGIGDDFFDY

SEQ ID NO: 461 - protein, 122 aa, synthetic construct
  REGION 1..122: note = source = /note="Description of Artificial Sequence: Synthetic polypeptide"
EVQLQQSGPELVKPGASMKISCKASGYSFTGYTMNWMKQGHGKNLEWIGLFNPYNGGPNYNQKFKGKATLTVDKSSSTAYMELLSLTSEDSAVYYCARLRYYGIGDDFFDYWGQGTTLTVSS

SEQ ID NO: 462 - protein, 11 aa, synthetic construct
  REGION 1..11: note = source = /note="Description of Artificial Sequence: Synthetic peptide"
KASQDVGTAVA

SEQ ID NO: 463 - protein, 7 aa, synthetic construct
  REGION 1..7: note = source = /note="Description of Artificial Sequence: Synthetic peptide"
WASTRHT

SEQ ID NO: 464 - protein, 9 aa, synthetic construct
  REGION 1..9: note = source = /note="Description of Artificial Sequence: Synthetic peptide"
QQYSSYPYT

SEQ ID NO: 465 - protein, 7 aa, synthetic construct
  REGION 1..7: note = source = /note="Description of Artificial Sequence: Synthetic peptide"
SQDVGTA

SEQ ID NO: 466 - skipped

SEQ ID NO: 467 - protein, 6 aa, synthetic construct
  REGION 1..6: note = source = /note="Description of Artificial Sequence: Synthetic peptide"
YSSYPY

SEQ ID NO: 468 - protein, 107 aa, synthetic construct
  REGION 1..107: note = source = /note="Description of Artificial Sequence: Synthetic polypeptide"
DIVMTQSHKFMSTSVGDRVSITCKASQDVGTAVAWYQQKPGQSPKLLIYWASTRHTGVPDRFTGSGSGTDFTLTITNVQSEDLTDYFCQQYSSYPYTFGGGTKLEIK

SEQ ID NO: 469 - protein, 5 aa, synthetic construct
  REGION 1..5: note = source = /note="Description of Artificial Sequence: Synthetic peptide"
GYTMN

SEQ ID NO: 470 - protein, 17 aa, synthetic construct
  REGION 1..17: note = source = /note="Description of Artificial Sequence: Synthetic peptide"
LFNPYNGGPSYNQKFKG

SEQ ID NO: 471 - protein, 13 aa, synthetic construct
  REGION 1..13: note = source = /note="Description of Artificial Sequence: Synthetic peptide"
LRYYGIGDDFFDY

SEQ ID NO: 472 - protein, 7 aa, synthetic construct
  REGION 1..7: note = source = /note="Description of Artificial Sequence: Synthetic peptide"
GYSFTGY

SEQ ID NO: 473 - protein, 6 aa, synthetic construct
  REGION 1..6: note = source = /note="Description of Artificial Sequence: Synthetic peptide"
NPYNGG

SEQ ID NO: 474 - protein, 13 aa, synthetic construct
  REGION 1..13: note = source = /note="Description of Artificial Sequence: Synthetic peptide"
LRYYGIGDDFFDY

SEQ ID NO: 475 - protein, 122 aa, synthetic construct
  REGION 1..122: note = source = /note="Description of Artificial Sequence: Synthetic polypeptide"
EVQLQQSGPDLVKPGASMKLSCKASGYSFTGYTMNWVKQSHGKNLEWIGLFNPYNGGPSYNQKFKGKATLTVDKSSSTAYMELLSLTPEDSAVYYCARLRYYGIGDDFFDYWGQGTTLTVSS

SEQ ID NO: 476 - protein, 11 aa, synthetic construct
  REGION 1..11: note = source = /note="Description of Artificial Sequence: Synthetic peptide"
KASQDVGTAVA

SEQ ID NO: 477 - protein, 7 aa, synthetic construct
  REGION 1..7: note = source = /note="Description of Artificial Sequence: Synthetic peptide"
WASTRHT

SEQ ID NO: 478 - protein, 9 aa, synthetic construct
  REGION 1..9: note = source = /note="Description of Artificial Sequence: Synthetic peptide"
QQYSNYPYT

SEQ ID NO: 479 - protein, 7 aa, synthetic construct
  REGION 1..7: note = source = /note="Description of Artificial Sequence: Synthetic peptide"
SQDVGTA

SEQ ID NO: 480 - skipped

SEQ ID NO: 481 - protein, 6 aa, synthetic construct
  REGION 1..6: note = source = /note="Description of Artificial Sequence: Synthetic peptide"
YSNYPY

SEQ ID NO: 482 - protein, 107 aa, synthetic construct
  REGION 1..107: note = source = /note="Description of Artificial Sequence: Synthetic polypeptide"
DIVMTQSHKFMSTSVGDRVSITCKASQDVGTAVAWYQEKPGQSPKLLIYWASTRHTGVPDRFTGSGSGTDFTLTISNVQSEDLAYYFCQQYSNYPYTFGGGTKLEIK

SEQ ID NO: 483 - protein, 5 aa, synthetic construct
  REGION 1..5: note = source = /note="Description of Artificial Sequence: Synthetic peptide"
GYTMN

SEQ ID NO: 484 - protein, 17 aa, synthetic construct
  REGION 1..17: note = source = /note="Description of Artificial Sequence: Synthetic peptide"
LFNPYNGGATYNQRFKG

SEQ ID NO: 485 - protein, 13 aa, synthetic construct
  REGION 1..13: note = source = /note="Description of Artificial Sequence: Synthetic peptide"
LRKYGIGDDFFDY

SEQ ID NO: 486 - protein, 7 aa, synthetic construct
  REGION 1..7: note = source = /note="Description of Artificial Sequence: Synthetic peptide"
GYSFTGY

SEQ ID NO: 487 - protein, 6 aa, synthetic construct
  REGION 1..6: note = source = /note="Description of Artificial Sequence: Synthetic peptide"
NPYNGG

SEQ ID NO: 488 - protein, 13 aa, synthetic construct
  REGION 1..13: note = source = /note="Description of Artificial Sequence: Synthetic peptide"
LRKYGIGDDFFDY

SEQ ID NO: 489 - protein, 122 aa, synthetic construct
  REGION 1..122: note = source = /note="Description of Artificial Sequence: Synthetic polypeptide"
EVQLQQSGPELVKPGASMKISCKASGYSFTGYTMNWVKQSHGKNLEWIGLFNPYNGGATYNQRFKGKATLTVDKSSSTAYMDLLSLTSEDSAVYYCTRLRKYGIGDDFFDYWGQGTTLTVSS

SEQ ID NO: 490 - protein, 11 aa, synthetic construct
  REGION 1..11: note = source = /note="Description of Artificial Sequence: Synthetic peptide"
KASQDVGTAVA

SEQ ID NO: 491 - protein, 7 aa, synthetic construct
  REGION 1..7: note = source = /note="Description of Artificial Sequence: Synthetic peptide"
WASTRHT

SEQ ID NO: 492 - protein, 9 aa, synthetic construct
  REGION 1..9: note = source = /note="Description of Artificial Sequence: Synthetic peptide"
QQYSTYTYT

SEQ ID NO: 493 - protein, 7 aa, synthetic construct
  REGION 1..7: note = source = /note="Description of Artificial Sequence: Synthetic peptide"
SQDVGTA

SEQ ID NO: 494 - skipped

SEQ ID NO: 495 - protein, 6 aa, synthetic construct
  REGION 1..6: note = source = /note="Description of Artificial Sequence: Synthetic peptide"
YSTYTY

SEQ ID NO: 496 - protein, 107 aa, synthetic construct
  REGION 1..107: note = source = /note="Description of Artificial Sequence: Synthetic polypeptide"
DIVMTQSHKFMSTSVGDRVSITCKASQDVGTAVAWYQQKPGQSPKLLIYWASTRHTGVPDRFTGSGSGTDFTLTISNVQSEDLADYFCQQYSTYTYTFGGGTKLEIK

SEQ ID NO: 497 - protein, 80 aa, synthetic construct
  REGION 1..80: note = source = /note="Description of Artificial Sequence: Synthetic polypeptide"
FSLKLSAENDFSSDSPERKMLPCYSTARIPLPNLNEDLTCGNLLMWEAVTVQTEVIGITSMLNLHAGSQKVHEHGGGKPI

SEQ ID NO: 498 - protein, 80 aa, synthetic construct
  REGION 1..80: note = source = /note="Description of Artificial Sequence: Synthetic polypeptide"
YSLKLTAENAFDSDSPDKKMLPCYSTARIPLPNLNEDLTCGNLLMWEAVTVKTEVIGITSMLNLHAGSQKVHENGGGKPV

SEQ ID NO: 499 - protein, 80 aa, synthetic construct
  REGION 1..80: note = source = /note="Description of Artificial Sequence: Synthetic polypeptide"
YSQHLSAENAFDSDSPDKKMLPCYSTARIPLPNLNEDLTCGNLLMWEAVTVKTEVIGITSMLNLHAGSQKVHENGGGKPV

SEQ ID NO: 500 - protein, 80 aa, synthetic construct
  REGION 1..80: note = source = /note="Description of Artificial Sequence: Synthetic polypeptide"
YSLRLTAETAFDSDSPDRKMLPCYSTARIPLPNLNEDLTCGNLLMWEAVTVKTEVIGITSMLNLHAGSQKVHENGGGKPI

SEQ ID NO: 501 - protein, 18 aa, synthetic construct
  MOD_RES 3: note = Any amino acid
  MOD_RES 5..6: note = Any amino acid
  VARIANT 7: note = /replace="Glu"
  SITE 7: note = MISC_FEATURE - /note="Variant residue given in the sequence has no preference with respect to that in the annotation for variant position"
  MOD_RES 8..12: note = Any amino acid
  MOD_RES 15: note = Any amino acid
  MOD_RES 17: note = Any amino acid
  REGION 1..18: note = source = /note="Description of Artificial Sequence: Synthetic peptide"
YRXKXXDXXXXXKNXTXQ

SEQ ID NO: 502 - protein, 23 aa, synthetic construct
  MOD_RES 8: note = Any amino acid
  MOD_RES 11..12: note = Any amino acid
  MOD_RES 16: note = Any amino acid
  MOD_RES 18: note = Any amino acid
  REGION 1..23: note = source = /note="Description of Artificial Sequence: Synthetic peptide"
NYRTKYPXGTXXPKNXTXQSQVM

SEQ ID NO: 503 - protein, 268 aa, synthetic construct
  REGION 1..268: note = source = /note="Description of Artificial Sequence: Synthetic polypeptide"
KGGVEVLEVKTGVDAITEVECFLNPEMGDPDENLRGFSLKLSAENDFSSDSPERKMLPCYSTARIPLPNLNEDLTCGNLLMWEAVTVQTEVIGITSMLNLHAGSQKVHEHGGGKPIQGSNFHFFAVGGDPLEMQGVLMNYRTKYPEGTITPKNPTAQSQVMNTDHKAYLDKNNAYPVECWIPDPSRNENTRYFGTFTGGENVPPVLHVTNTATTVLLDEQGVGPLCKADSLYVSAADICGLFTNSSGTQQWRGLARYFKIRLRKRSVK

SEQ ID NO: 504 - protein, 268 aa, synthetic construct
  REGION 1..268: note = source = /note="Description of Artificial Sequence: Synthetic polypeptide"
KGGVEVLEVKTGVDAITEVECFLNPEMGDPDDNLRGYSLKLTAENAFDSDSPDKKMLPCYSTARIPLPNLNEDLTCGNLLMWEAVTVKTEVIGITSMLNLHAGSQKVHENGGGKPVQGSNFHFFAVGGDPLEMQGVLMNYRTKYPQGTITPKNPTAQSQVMNTDHKAYLDKNNAYPVECWIPDPSRNENTRYFGTYTGGENVPPVLHVTNTATTVLLDEQGVGPLCKADSLYVSAADICGLFTNSSGTQQWRGLARYFKIRLRKRSVK

SEQ ID NO: 505 - protein, 268 aa, synthetic construct
  REGION 1..268: note = source = /note="Description of Artificial Sequence: Synthetic polypeptide"
KGGVEVLEVKTGVDAITEVECFLNPEMGDPDDHLRGYSQHLSAENAFDSDSPDKKMLPCYSTARIPLPNLNEDLTCGNLLMWEAVTVKTEVIGITSMLNLHAGSQKVHENGGGKPVQGSNFHFFAVGGDPLEMQGVLMNYRTKYPQGTITPKNPTAQSQVMNTDHKAYLDKNNAYPVECWIPDPSKNENTRYFGTYTGGENVPPVLHVTNTATTVLLDEQGVGPLCKADSLYVSAADICGLFTNSSGTQQWRGLARYFKIRLRKRSVK

SEQ ID NO: 506 - protein, 268 aa, synthetic construct
  REGION 1..268: note = source = /note="Description of Artificial Sequence: Synthetic polypeptide"
KGGVEVLEVKTGVDAITEVECFLNPEMGDPDNDLRGYSLRLTAETAFDSDSPDRKMLPCYSTARIPLPNLNEDLTCGNLLMWEAVTVKTEVIGITSMLNLHAGSQKVHENGGGKPIQGSNFHFFAVGGDPLEMQGVLMNYRTKYPEGTVTPKNPTAQSQVMNTDHKAYLDKNNAYPVECWIPDPSRNENTRYFGTYTGGENVPPVLHVTNTATTVLLDEQGVGPLCKADSLYVSAADICGLFTNSSGTQQWRGLPRYFKIRLRKRSVK

SEQ ID NO: 507 - protein, 6 aa, synthetic construct
  REGION 1..6: note = source = /note="Description of Artificial Sequence: Synthetic 6xHis tag"
HHHHHH

SEQ ID NO: 508 - protein, 10 aa, synthetic construct
  MOD_RES 5: note = Any amino acid
  REGION 1..10: note = source = /note="Description of Artificial Sequence: Synthetic polypeptide"
GFTFXNYWMT

SEQ ID NO: 509 - protein, 10 aa, synthetic construct
  REGION 1..10: note = source = /note="Description of Artificial Sequence: Synthetic peptide"
GFTFNNYWMT

SEQ ID NO: 510 - protein, 17 aa, synthetic construct
  REGION 1..17: note = source = /note="Description of Artificial Sequence: Synthetic peptide"
NIKKDGSEKYYVDSVRG

SEQ ID NO: 511 - protein, 44 aa, synthetic construct
  REGION 1..44: note = source = /note="Description of Artificial Sequence: Synthetic peptide"
  REGION 1..44: note = source = /note="Description of Artificial Sequence: Synthetic peptide"
VALARGSERGLYARGTYRPHEALALEUASPASPGGDNIGSRPVH

SEQ ID NO: 512 - protein, 7 aa, synthetic construct
  REGION 1..7: note = source = /note="Description of Artificial Sequence: Synthetic peptide"
DDSNRPS

SEQ ID NO: 513 - protein, 10 aa, synthetic construct
  REGION 1..10: note = source = /note="Description of Artificial Sequence: Synthetic peptide"
QVWSSSTDHP

SEQ ID NO: 514 - protein, 10 aa, synthetic construct
  REGION 1..10: note = source = /note="Description of Artificial Sequence: Synthetic peptide"
GFTFSNYWMT

SEQ ID NO: 515 - protein, 17 aa, synthetic construct
  REGION 1..17: note = source = /note="Description of Artificial Sequence: Synthetic peptide"
NIKKDGSEKYYVDSVRG

SEQ ID NO: 516 - protein, 44 aa, synthetic construct; identical to SEQ ID NO: 511
  REGION 1..44: note = source = /note="Description of Artificial Sequence: Synthetic peptide"
  REGION 1..44: note = source = /note="Description of Artificial Sequence: Synthetic peptide"

SEQ ID NO: 517 - protein, 7 aa, synthetic construct
  REGION 1..7: note = source = /note="Description of Artificial Sequence: Synthetic peptide"
DDSNRPS

SEQ ID NO: 518 - protein, 10 aa, synthetic construct
  REGION 1..10: note = source = /note="Description of Artificial Sequence: Synthetic peptide"
QVWSSSTDHP

SEQ ID NO: 519 - protein, 10 aa, synthetic construct
  REGION 1..10: note = source = /note="Description of Artificial Sequence: Synthetic peptide"
GFTFKNYWMT

SEQ ID NO: 520 - protein, 17 aa, synthetic construct
  REGION 1..17: note = source = /note="Description of Artificial Sequence: Synthetic peptide"
NIKKDGSEKYYVDSVRG

SEQ ID NO: 521 - protein, 44 aa, synthetic construct; identical to SEQ ID NO: 511
  REGION 1..44: note = source = /note="Description of Artificial Sequence: Synthetic peptide"
  REGION 1..44: note = source = /note="Description of Artificial Sequence: Synthetic peptide"

SEQ ID NO: 522 - protein, 7 aa, synthetic construct
  REGION 1..7: note = source = /note="Description of Artificial Sequence: Synthetic peptide"
DDSNRPS

SEQ ID NO: 523 - protein, 10 aa, synthetic construct
  REGION 1..10: note = source = /note="Description of Artificial Sequence: Synthetic peptide"
QVWSSSTDHP

SEQ ID NO: 524 - protein, 10 aa, synthetic construct
  REGION 1..10: note = source = /note="Description of Artificial Sequence: Synthetic peptide"
GFTFQNYWMT

SEQ ID NO: 525 - protein, 17 aa, synthetic construct
  REGION 1..17: note = source = /note="Description of Artificial Sequence: Synthetic peptide"
NIKKDGSEKYYVDSVRG

SEQ ID NO: 526 - protein, 44 aa, synthetic construct; identical to SEQ ID NO: 511
  REGION 1..44: note = source = /note="Description of Artificial Sequence: Synthetic peptide"
  REGION 1..44: note = source = /note="Description of Artificial Sequence: Synthetic peptide"

SEQ ID NO: 527 - protein, 7 aa, synthetic construct
  REGION 1..7: note = source = /note="Description of Artificial Sequence: Synthetic peptide"
DDSNRPS

SEQ ID NO: 528 - protein, 10 aa, synthetic construct
  REGION 1..10: note = source = /note="Description of Artificial Sequence: Synthetic peptide"
QVWSSSTDHP

SEQ ID NO: 529 - protein, 10 aa, synthetic construct
  REGION 1..10: note = source = /note="Description of Artificial Sequence: Synthetic peptide"
GFTFNNYWMT

SEQ ID NO: 530 - protein, 17 aa, synthetic construct
  REGION 1..17: note = source = /note="Description of Artificial Sequence: Synthetic peptide"
NIKKDGSEKYYVDSVRG

SEQ ID NO: 531 - protein, 44 aa, synthetic construct; identical to SEQ ID NO: 511
  REGION 1..44: note = source = /note="Description of Artificial Sequence: Synthetic peptide"
  REGION 1..44: note = source = /note="Description of Artificial Sequence: Synthetic peptide"

SEQ ID NO: 532 - protein, 7 aa, synthetic construct
  REGION 1..7: note = source = /note="Description of Artificial Sequence: Synthetic peptide"
DDSNRPS

SEQ ID NO: 533 - protein, 10 aa, synthetic construct
  REGION 1..10: note = source = /note="Description of Artificial Sequence: Synthetic peptide"
QVWSSSTDHP

SEQ ID NO: 534 - protein, 10 aa, synthetic construct
  REGION 1..10: note = source = /note="Description of Artificial Sequence: Synthetic peptide"
GFTFNNYWMT

SEQ ID NO: 535 - protein, 17 aa, synthetic construct
  REGION 1..17: note = source = /note="Description of Artificial Sequence: Synthetic peptide"
NIKKDGSEKYYVDSVRG

SEQ ID NO: 536 - protein, 44 aa, synthetic construct; identical to SEQ ID NO: 511
  REGION 1..44: note = source = /note="Description of Artificial Sequence: Synthetic peptide"
  REGION 1..44: note = source = /note="Description of Artificial Sequence: Synthetic peptide"

SEQ ID NO: 537 - protein, 7 aa, synthetic construct
  REGION 1..7: note = source = /note="Description of Artificial Sequence: Synthetic peptide"
DDSNRPS

SEQ ID NO: 538 - protein, 10 aa, synthetic construct
  REGION 1..10: note = source = /note="Description of Artificial Sequence: Synthetic peptide"
QVWSSSTDHP